European Patent Specification EP 3 585 162 B1, published August 30, 2023. Title: NON-HUMAN ANIMALS COMPRISING A HUMANIZED TTR LOCUS AND METHODS OF USE. Applicant: Regeneron Pharmaceuticals, Inc. The sequence listing filed with the application follows.

SEQUENCE LISTING (94 sequences)

SEQ ID NO: 1 - protein, 147 aa, Homo sapiens
MASHRLLLLCLAGLVFVSEAGPTGTGESKCPLMVKVLDAVRGSPAINVAVHVFRKAADDTWEPFASGKTSESGELHGLTTEEEFVEGIYKVEIDTKSYWKALGISPFHEHAEVVFTANDSGPRRYTIAALLSPYSYSTTAVVTNPKE

SEQ ID NO: 2 - protein, 147 aa, Artificial Sequence
  Synthetic
MASLRLFLLCLAGLVFVSEAGPAGTGESKCPLMVKVLDAVRGSPAINVAVHVFRKAADDTWEPFASGKTSESGELHGLTTEEEFVEGIYKVEIDTKSYWKALGISPFHEHAEVVFTANDSGPRRYTIAALLSPYSYSTTAVVTNPKE

SEQ ID NO: 3 - DNA, 7258 bp, Homo sapiens
gttgactaagtcaataatcagaatcagcaggtttgcagtcagattggcagggataagcagcctagctcaggagaagtgagtataaaagccccaggctgggagcagccatcacagaagtccactcattcttggcaggatggcttctcatcgtctgctcctcctctgccttgctggactggtatttgtgtctgaggctggccctacggtgagtgtttctgtgacatcccattcctacatttaagattcacgctaaatgaagtagaagtgactccttccagctttgccaaccagcttttattactagggcaagggtacccagcatctatttttaatataattaattcaaacttcaaaaagaatgaagttccactgagcttactgagctgggacttgaactctgagcattctacctcattgctttggtgcattaggtttgtaatatctggtacctctgtttcctcagatagatgatagaaataaagatatgatattaaggaagctgttaatactgaattttcagaaaagtatccctccataaaatgtatttgggggacaaactgcaggagattatattctggccctatagttattcaaaacgtatttattgattaatctttaaaaggcttagtgaacaatattctagtcagatatctaattcttaaatcctctagaagaattaactaatactataaaatgggtctggatgtagttctgacattattttataacaactggtaagagggagtgactatagcaacaactaaaatgatctcaggaaaacctgtttggccctatgtatggtacattacatcttttcagtaattccactcaaatggagacttttaacaaagcaactgttctcaggggacctattttctcccttaaaattcattatacacatccctggttgatagcagtgtgtctggaggcagaaaccattcttgctttggaaacaattacgtctgtgttatactgagtagggaagctcattaattgtcgacacttacgttcctgataatgggatcagtgtgtaattcttgtttcgctccagatttctaataccacaaagaataaatcctttcactctgatcaattttgttaacttctcacgtgtcttctctacacccagggcaccggtgaatccaagtgtcctctgatggtcaaagttctagatgctgtccgaggcagtcctgccatcaatgtggccgtgcatgtgttcagaaaggctgctgatgacacctgggagccatttgcctctgggtaagttgccaaagaaccctcccacaggacttggttttatcttcccgtttgcccctcacttggtagagagaggctcacatcatctgctaaagaatttacaagtagattgaaaaacgtaggcagaggtcaagtatgccctctgaaggatgccctctttttgttttgcttagctaggaagtgaccaggaacctgagcatcatttaggggcagacagtagagaaaagaaggaatcagaactcctctcctctagctgtggtttgcaacccttttgggtcacagaacactttatgtaggtgatgaaaagtaaacattctatgcccagaaaaaatgcacagatacacacacatacaaaatcatatatgtgattttaggagtttcacagattccctggtgtccctgggtaacaccaaagctaagtgtccttgtcttagaattttaggaaaaggtataatgtgtattaacccattaacaaaaggaaaggaattcagaaatattattaaccaggcatctgtctgtagttaatatggatcacccaaaacccaaggcttttgcctaatgaacactttggggcacctactgtgtgcaaggctgggggctgtcaagctcagttaaaaaaaaaaagatagaagagatggatccatgaggcaaagtacagccccaggctaatcccacgatcacccgacttcatgtccaagagtggcttctcaccttcattagccagttcacaattttcatggagtttttctacctgcactagcaaaaacttcaaggaaaatacatattaataaatctaagcaaagtgaccagaagacagagcaatcaggagaccctttgcatccagcagaagaggaactgctaagtatttacatctccacagagaagaatttctgttgggttttaattgaaccccaagaaccacatgattcttcaaccattattgggaagatcattttcttaggtctggttttaactggctttttatttgggaattcatttatgtttatataaaatgccaagcataacatgaaaagtggttacaggactattctaagggagagacagaatggacaccaaaaatattccaatgttcttgtgaatcttttccttgcaccaggacaaaaaaaaaaagaagtgaaaagaagaaaggaggaggggcataatcagagtcagtaaagacaactgctatttttatctatcgtagctgttgcagtcaaatgggaagcaatttccaacattcaactatggagctggtacttacatggaaatagaagttgcctagtgtttgttgctggcaaagagttatcagagaggttaaatatataaaagggaaaagagtcagatacaggttcttcttcctactttaggttttccactgtgtgtgcaaatgatactccctggtggtgtgcagatgcctcaaagctatcctcacaccacaagggagaggagcgagatcctgctgtcctggagaagtgcagagttagaacagctgtggccacttgcatccaatcatcaatcttgaatcacagggactctttcttaagtaaacattatacctggccgggcacggtggctcacgcctgtaatcccagcactttgggatgccaaagtgggcatatcatctgaggtcaggagttcaagaccagcctggccaacatggcaaaactccgtctttatgaaaaatacaaaaattagccaggcatggtggcaggcgcctgtaatcccagctaattgggaggctgaggctggagaatcccttgaatctaggaggcagaggttgcagtgagctgagatcgtgccattgcactccagcctgggtgacaagagtaaaactctgtctcaaaaaaaaaaaattatacctacattctcttcttatcagagaaaaaaatctacagtgagcttttcaaaaagtttttacaaactttttgccatttaatttcagttaggagttttccctacttctgacttagttgaggggaaatgttcataacatgtttataacatgtttatgtgtgttagttggtgggggtgtattactttgccatgccatttgtttcctccatgcgtaacttaatccagactttcacaccttataggaaaaccagtgagtctggagagctgcatgggctcacaactgaggaggaatttgtagaagggatatacaaagtggaaatagacaccaaatcttactggaaggcacttggcatctccccattccatgagcatgcagaggtgagtatacagaccttcgagggttgttttggttttggtttttgcttttggcattccaggaaatgcacagttttactcagtgtaccacagaaatgtcctaaggaaggtgatgaatgaccaaaggttccctttcctattatacaagaaaaaattcacaacactctgagaagcaaatttctttttgactttgatgaaaatccacttagtaacatgacttgaacttacatgaaactactcatagtctattcattccactttatatgaatattgatgtatctgctgttgaaataatagtttatgaggcagccctccagaccccacgtagagtgtatgtaacaagagatgcaccattttatttctcgaaaacccgtaacattcttcattccaaaacacatctggcttctcggaggtctggacaagtgattcttggcaacacatacctatagagacaataaaatcaaagtaataatggcaacacaatagataacatttaccaagcatacaccatgtggcagacacaattataagtgttttccatatttaacctacttaatcctcaggaataagccactgaggtcagtcctattattatccccatcttatagatgaagaaaatgaggcaccaggaagtcaaataacttgtcaaaggtcacaagactaggaaatacacaagtagaaatgtttacaattaaggcccaggctgggtttgccctcagttctgctatgcctcgcattatgccccaggaaactttttcccttgtgaaagccaagcttaaaaaaagaaaagccacatttgtaacgtgctctgttcccctgcctatggtgaggatcttcaaacagttatacatggacccagtccccctgccttctccttaatttcttaagtcatttgaaacagatggctgtcatggaaatagaatccagacatgttggtcagagttaaagatcaactaattccatcaaaaatagctcggcatgaaagggaactattctctggcttagtcatggatgagactttcaattgctataaagtggttcctttattagacaatgttaccagggaaacaacaggggtttgtttgacttctggggcccacaagtcaacaagagagccccatctaccaaggagcatgtccctgactacccctcagccagcagcaagacatggaccccagtcagggcaggagcagggtttcggcggcgcccagcacaagacattgcccctagagtctcagcccctaccctcgagtaatagatctgcctacctgagactgttgtttgcccaagagctgggtctcagcctgatgggaaccatataaaaaggttcactgacatactgcccacatgttgttctctttcattagatcttagcttccttgtctgctcttcattcttgcagtattcattcaacaaacattaaaaaaaaaaaaaagcattctatgtgtggaacactctgctagatgctgtggatttagaaatgaaaatacatcccgacccttggaatggaagggaaaggactgaagtaagacagattaagcaggaccgtcagcccagcttgaagcccagataaatacggagaacaagagagagcgagtagtgagagatgagtcccaatgcctcactttggtgacgggtgcgtggtgggcttcatgcagcttcttctgataaatgcctccttcagaactggtcaactctaccttggccagtgacccaggtggtcatagtagatttaccaagggaaaatggaaacttttattaggagctcttaggcctcttcacttcatggatttttttttcctttttttttgagatggagttttgccctgtcacccaggctggaatgcagtggtgcaatctcagctcactgcaacctccgcctcccaggttcaagcaattctcctgcctcagcctcccgagtagctgggactacaggtgtgcgccaccacaccaggctaatttttgtattttttgtaaagacaggttttcaccacgttggccaggctggtctgaactccagacctcaggtgattcacctgtctcagcctcccaaagtgctgggattacaggtgtgagccaccgtgcccggctacttcatggatttttgattacagattatgcctcttacaatttttaagaagaatcaagtgggctgaaggtcaatgtcaccataagacaaaagacatttttattagttgattctagggaattggccttaaggggagccctttcttcctaagagattcttaggtgattctcacttcctcttgccccagtattatttttgtttttggtatggctcactcagatccttttttcctcctatccctaagtaatccgggtttctttttcccatatttagaacaaaatgtatttatgcagagtgtgtccaaacctcaacccaaggcctgtatacaaaataaatcaaattaaacacatctttactgtcttctacctctttcctgacctcaatatatcccaacttgcctcactctgagaaccaaggctgtcccagcacctgagtcgcagatattctactgatttgacagaactgtgtgactatctggaacagcattttgatccacaatttgcccagttacaaagcttaaatgagctctagtgcatgcatatatatttcaaaattccaccatgatcttccacactctgtattgtaaatagagccctgtaatgcttttacttcgtatttcattgcttgttatacataaaaatatacttttcttcttcatgttagaaaatgcaaagaataggagggtgggggaatctctgggcttggagacaggagacttgccttcctactatggttccatcagaatgtagactgggacaatacaataattcaagtctggtttgctcatctgtaaattgggaagaatgtttccagctccagaatgctaaatctctaagtctgtggttggcagccactattgcagcagctcttcaatgactcaatgcagttttgcattctccctaccttttttttctaaaaccaataaaatagatacagcctttaggctttctgggatttcccttagtcaagctagggtcatcctgactttcggcgtgaatttgcaaaacaagacctgactctgtactcctgctctaaggactgtgcatggttccaaaggcttagcttgccagcatatttgagctttttccttctgttcaaactgttccaaaatataaaagaataaaattaattaagttggcactggacttccggtggtcagtcatgtgtgtcatctgtcacgtttttcgggctctggtggaaatggatctgtctgtcttctctcataggtggtattcacagccaacgactccggcccccgccgctacaccattgccgccctgctgagcccctactcctattccaccacggctgtcgtcaccaatcccaaggaatgagggacttctcctccagtggacctgaaggacgagggatgggatttcatgtaaccaagagtattccatttttactaaagcagtgttttcacctcatatgctatgttagaagtccaggcagagacaataaaacattcctgtgaaaggcacttttcattccactttaacttgattttttaaattcccttattgtcccttccaaaaaaaagagaatcaaaattttacaaagaatcaaaggaattctagaaagtatctgggcagaacgctaggagagatccaaatttccattgtcttgcaagcaaagcacgtattaaatatgatctgcagccattaaaaagacacattctgtaaa

SEQ ID NO: 4 - DNA, 938 bp, Homo sapiens
gttgactaagtcaataatcagaatcagcaggtttgcagtcagattggcagggataagcagcctagctcaggagaagtgagtataaaagccccaggctgggagcagccatcacagaagtccactcattcttggcaggatggcttctcatcgtctgctcctcctctgccttgctggactggtatttgtgtctgaggctggccctacgggcaccggtgaatccaagtgtcctctgatggtcaaagttctagatgctgtccgaggcagtcctgccatcaatgtggccgtgcatgtgttcagaaaggctgctgatgacacctgggagccatttgcctctgggaaaaccagtgagtctggagagctgcatgggctcacaactgaggaggaatttgtagaagggatatacaaagtggaaatagacaccaaatcttactggaaggcacttggcatctccccattccatgagcatgcagaggtggtattcacagccaacgactccggcccccgccgctacaccattgccgccctgctgagcccctactcctattccaccacggctgtcgtcaccaatcccaaggaatgagggacttctcctccagtggacctgaaggacgagggatgggatttcatgtaaccaagagtattccatttttactaaagcagtgttttcacctcatatgctatgttagaagtccaggcagagacaataaaacattcctgtgaaaggcacttttcattccactttaacttgattttttaaattcccttattgtcccttccaaaaaaaagagaatcaaaattttacaaagaatcaaaggaattctagaaagtatctgggcagaacgctaggagagatccaaatttccattgtcttgcaagcaaagcacgtattaaatatgatctgcagccattaaaaagacacattctgtaaaaaaaaaaaa

SEQ ID NO: 5 - DNA, 9077 bp, Mus musculus
ctaatctccctaggcaaggttcatatttgtgtaggttacttattctccttttgttgactaagtcaataatcagaatcagcaggtttggagtcagcttggcagggatcagcagcctgggttggaaggagggggtataaaagccccttcaccaggagaagccgtcacacagatccacaagctcctgacaggatggcttcccttcgactcttcctcctttgcctcgctggactggtatttgtgtctgaagctggccccgcggtgagtgatcctgtgagcgatccagacatggcagttagaccttagataaagaagaagtgccttcttccagatgtgagaactagagtactcagactctatatttaccattagactccaaagagaagagctggagtgcctctggctcttccttctattgctttagcgcattgggtctgtagtgctcagtctctggtgtccttagataataaagatatgagattaacatagaaataaagatataaaagggctggatgtatagtttagtggtccagtgtatgcctagtatgtgaaaagccttctgttcaacctctagcaatagaaaaacaagatatattctcggtggggctgttaatattgaattctcataaaatctttaatatatttagtatgcctattatgttgttatattttagttctttagctaatcaaaatgcattattgatctttctttgtctttttttggccaacactctattccagtctttgaaaaagtcctttaaaagagttaatcagtataattaaatgagtcaggaagtatgtgagggttattttacaaccagagggaattactatagcaacagctgattagaatgatctcaagaaaaagcccattctgtctttttgcaccatgcacctttcagtggctccattcagatggagaggcaaacagagcaatggctctcagagggcctattttccctttgaacattcattatccatatccctggtgcacagcagtgcatctgggggcagaaactgttcttgctttggaaacaatgctgtctatgtcatactggataaagaagctcattaattgtcaacacttatgttatcataatgggatcagcatgtacttttggttttgttccagagtctatcaccggaaagaacaagccggtttactctgacccatttcactgacatttctcttgtctcctctgtgcccagggtgctggagaatccaaatgtcctctgatggtcaaagtcctggatgctgtccgaggcagccctgctgtagacgtggctgtaaaagtgttcaaaaagacctctgagggatcctgggagccctttgcctctgggtaagcttgtagaaagcccaccatgggaccggttccaggttcccatttgctcttattcgtgttagattcagacacacacaacttaccagctagagggctcagagagagggctcaggggcgaagggcacgtattgctcttgtaagagacacaggtttaattcctagcaccagaatggcagctcataaccatctgaaactcacagtcttaggagatctgggtatctgacattctcttctacccaccatgtgtgtggtgcacaaattcacatgcaggcatcaaatcttataaacaacaacaaaaaaccaacaaacctggtagcaaaagaagattagaaggttaaacatatgagccgagagcttttgttttgttttgttttgttttgttttgtttacatttcaaatgttatcccctttctcggtccccctccccaaaccctctaccccattctctcctccccttcttctatgagggtgttccccaccaacccactcccaccttcctgctctcgaattcccctatactgggacatcaagccttcacagaatcaagggcctctcctcccattgatgcccgacaatgtcatcctctgctacctatgtggctggagccatgggtcccttcatgtatcctccttggttggtggtttagtctctgggaggtctgggggatctggttgattgatattattgttcttcctatgagattgcaaaccccttcagctccttcggtcctttaactcctccactggggaccccgagctcagtccaatggttggctgtgagcatccaccagcagaggcctttttttttttttttaacaaagctgctttattatgttgcttagagcatgaccaggaaccagagcacagtccaagactgaagggaggaaaagggggggagtcaataaccccactgtttcatagtggtttgcaacccttttatatcacagcccactttaggcaaataatgaaaattatagtctccagggacagagaagatggtgcaggaagtgaagtgcctgctcagaaaatgggggcttgaatgtgagttcccagactctgtgtaagatgcccagcatcgaagtgcatgcttataacaccagcctggaggtagaagcttagaaacaggggtaccctgaagttgcttgttcaccagtgtccctgaatgggtaggtgcatgtttggtgagagaccctgtctcaaaaatcaaggtgtaggataattgaaaatacctagctttgagcttagatcatgcaaatgtgtacacacactcacacacaccacacacacaaaaaaatgcagagacagagagatacagagagacagagagatacagagacagagacagagagaaaaggagaaagtaaaaaacaaataatttaaagacccatggccacaaagaggctcaaagacaagcacgtataaaaccatacacatgtaattttaggagttttcagattccctggtacccgtgggtgatgcacaagctttgaatcccagtcttaaaatcttacgaagaacgtgttcgtgtgtgctaatttattgatgagaggaaaggaattgacaaagtgcccttccggagcttcctgcattacccagactcagggtttttttaaatgtacactcagaacagagtagctctgtgcaagggtagcaaccacgaagcttaataagaaacatatcgtgagagatctgcaaggcaaatctaggggctgaccaatctcacagtcacccactagcatgtcaacacaacttcccacctgtgctagccacttagcaattttgtgttgttctgttttgtttttgtttttaacaaagcaatttcaaagagatttctaattcatctaaacaaacaaaccaaaaggaaaacagcaaagacgccctgagcacttagcagagcagctatgcagttatgactcctgggtggagactttatatcaggcttcaactgaatacctagaacctactagtgctcttcatcaatccttgggaaggtcattttcttttggtgctgttttgagtttctatttgttaatgtcttcataattatacacgtgttgagcacagcatgcaaagtgattaggggaatctagttggagtggaatggatacccaaatattcagactttcttgtgactcttctttcttgtacccacatcaaaaaaaaaaaaaatggagatgagacatggtcagagtcactaaaaccagctgctacttttaattacgtggggagcagtttctaacattgccattattgaactgatgctgcctgggtggaaatggaaatcacttagtatttcttgttggcaaagaattactgaatggattaaatttccaaagggagaagtcagttacaagtcttttctttgtttattaggctttctgctatgataaattacactacttccagaagttacccttaggccatgggacactggactatcactctgctgtcacaagagattacagagttagtcaaggcagcttgtgacaccttcagggactgtcataaacttccagcaagtcattaatcctgaatgcaatactgtgtgtgtgtgtctatgtgtgtttgtatgtctgtgtgtgtcttatgtctgtgtctctgtgtgtgtgtgtgtttgtgtgtgtgtgtgtatgtatgcctgtgtgtgtcttatgtctgtgtttgtgtgtctgtgtgtgtcttatgtctgtgtttgtatgtctgtgtgtgtctgtgtgtgtcttatgtctgtgtctctgtgtgtgtgtgtgtgtatgtatgtatgtatgtatgtatgtgtatgtgtttgcatctctctgtgtgtctgcgcttatatatttgtgtatgtgtttatgtgttcgcctttgtgcgttgttggggattgaatccaggggaatacaaatgttaagaaagaacgttaccactaagcttcacctgtaggccttaaagcttttctttcttttaaaaattgtaattaattcattttcagtcaggatctccacacctcgtccctgctgctctagaactcactatttaaacacaatcgccctcaaacctgcagcaaccctcccgcctctaccctgcgagcactagaataataacaggtgaccccacacgcctagattaagacctttaaggtaaacattttactatattttagtctcataagacaagatgctacaataaagctgtacataaagttccctcgaatttcttgctattttaactcaaacataaggatttcctcctttttgattcaggtaacagaaaaaatacacaggtacatacatgtacacacatgaacacacacgcatcacaaccacatatgcgcacgcttgtgtgatctatcatttaccatgccactgaactcttctttccccataaattcctctggacttgtgtgccctccaggaagaccgcggagtctggagagctgcacgggctcaccacagatgagaagtttgtagaaggagtgtacagagtagaactggacaccaaatcgtactggaagacacttggcatttccccgttccatgaattcgcggatgtaagtggacacaccaagttgtttggattttgtttttagtctcaggaaattcccttcgctcttgctgtacgatgggcatgagtggaaagtagattccacagccagaatccacagtgctgggaaagcaagccttctgaatttttctaaaactcatttagcaacatggcctgaacctgttcacactgcttatggtcagctaactatatttatgtaaatattcatttctctgttgaggaaatgttagtatttgcttttgaggcaacctccagataccatggagggcatgtcatagtcaaagagagggctccctatggtatttctctaaattctggcatttcctttattccaaagcacatctagtgtccccagaagtttgggtagacaattcttggcaacacagagaattacaacatgttcaaaacccaacagcttaatatctaaatcatcaagcaaacatcacatggcaaagggatttctgaatcaaaactgtttcatccttatgatcaacctatggaggtctagcctcgacttacacccattttaccaataagctaagagaagctaagttcctcatcaaggacacaaggctagcatgtgtgagcaagtgacagagttgccctctatgttggttagtgtgccttagccagtgtctcagtaagaaatggagctaaatcaaaacccaaggccaacagccaaaggcacatgagtaacctttgcttggcactgggctcagtttccctggctcctctcagtcctcagttcacagaggcagctgtcatgcaaatagaatccaagcttgttggtcagacctggagataacaaattccatcaaaaatagctcctcatgtgacctagtttgctgtctgttgctatgatacacaccatgaccgaaaagcaaccctggggagagaagggtttatttcatcttacagcttacagttcaccatggaggaaagccaggtgggaacctggaagtggaaattgaagcagagaccagaaaggaatgctgtttactggctggcttagctccttttcttatacagcttaggtctatgtgcccaggggatggtactgccgagcataggctgagcccgcctacatcaaccattagtcaaaaaaaggtccatagacttgcctacaggccaatctcatggaggcaataccccagtggagggtccctcttcgcaggttactctagtttgtgtcaagttgacaaaacctaaccacaaagcacaaacagggtctgcccttgtggcttagccatggatgacactctcagatgatggtgttaccagacaaaccagaggggctcaccaagagtctgccacctaccaaggtagtactctactcctcactgggcaccaacacccatattagctgggccagtacaggacccttgctgtttcctgcatgaattgtccatagaccctgggtctcagcctgccgggagtacctgtaagtagtcgcctcaaacacattattcctgttggaagacttgtctgattctcttttagaactcaatcaacaaacgtttttattttgttttggctttttggagacaagatctctcataggccagcctgacttgaatgtagctgaggatgacctgtgctgctaatcttctcgcctcttcctcccaagtggtaggataataggcataagacaccacagcagttttactccataccagggctctgaacccagactttaaacactctatcaactgattcacattcccaccccatcattcaacaaacatttgaaaaataaaacccttctgccttgagcactctgctaaatacagcctttgagtgcggagtatttcctcacaaccagggtccaagatgaccccatcatacataccacggaaaattaggagatgtttttaggtctctttgcttggggtaatttttatgtgtgtgtgtacacagccctgtgcgtgtgtgtgtgtgtgtgtgtgtgtgtgtacaggcacacacgtgtatgcatgtagaggctacataaaaaccttaggtgtcattctcaggcactctgttcaccccttcacacagcccgaacacacaaaatttgaggcattagcctggagctcaccagttaggctagactgacttgccagcagaccccaggctgtctccatctccccagctctgggattacaaactctatcataccagacatttttatacatattctgagcataaaattcatgtcttcaggctaacaagtcaagagcttaaatgactgagctctcttacgtggtggattttttttaaaactacataatatcttttttttttttttcacttctggggaagaaacaaatgagcctgagtgacaatgcgacagaaaagaaattttgaggagtgtgtgtgtctgtgtgtgtggtggcacatgcctctcatctaatgctagaggctacagtagaatgctcctgaattagtggccagccaaggccaagggctagggttgtaactcagtggcagagggcttgcctagcattcgcaggatttgatccatagcgctataaataataataaataaatacaacagtctaagatgattctccctttcatttatctggatgttatttttgtgttagttttactctgtcatccaatcattgtttgccctatatttggacatttaaaaaaaatctttattccaagtgtgttcaaagctgtatccaaaacctgtccaccaaatgagtccaatgacatacatcttctatattaccatctgttccagatttggctgactcccggcacctgggctgttgctgcacccatgtctcagatagtctagtgatttgagaagtgactagtaattgcaaaatccagactttgtccagaaacttctatgagctccaaaactttcatttacatttctgccagccacaaaccgcttgtgttgtggagagaaccctgtgatgtcttcccacagcatctcagccttgtttcttcccttaaaatattcatcttttcacattagaacatgcaaagggacagtgggagcgaaacccctggactgggacgcacgaagccttcctttctggtcaggctctcactgtagaaacttaggccggtttcagcatgcagtctgctggagaatggctcctgccaacattccaggtctggaagtttgtagtggagttgttgataaccactgttcgccacaggtcttttgtttgtgggtgtcagtgtttctactctcctgacttttatctgaacccaagaaagggaacaatagccttcaagctctctgtgactctgatctgaccagggccacccacactgcagaaggaaacttgcaaagagagacctgcaattctctaagagctccacacagctccaaagacttaggcagcatattttaatctaattattcgtcccccaaccccaccccagaggacagttagacaataaaaggaagattaccagcttagcatcctgtgaacactttgtctgcagctcctacctctgggctctgttagaactagctgtctctcctctctcctaggtggttttcacagccaacgactctggccatcgccactacaccatcgcagccctgctcagcccatactcctacagcaccacggctgtcgtcagcaacccccagaattgagagactcagcccaggaggaccaggatcttgccaaagcagtagcatcccatttgtaccaaaacagtgttcttgctctataaaccgtgttagcagctcaggaagatgccgtgaagcattcttattaaaccacctgctatttcattcaaactgtgtttcttttttatttcctcatttttctcccctgctcctaaaacccaaaatcttctaaagaattctagaaggtatgcgatcaaactttttaaagaaagaaaatactttttgactcatggtttaaaggcatcctttccatcttggggaggtcatgggtgctcctggcaacttgcttgaggaagataggtcagaaagcagagtggaccaaccgttcaatgttttacaagcaaaacatacactaagcatggtctgtagctattaaaagcacacaatctgaagggctgtagatgcacagtagtgttttcccagagcatgttcaaaagccctgggttcaatcacaatactgaaaagtaggccaaaaaacattctgaaaatgaaatatttgggtttttttttataacctttagtgactaaataaagacaaatctaagagactaa

SEQ ID NO: 6 - protein, 147 aa, Mus musculus
MASLRLFLLCLAGLVFVSEAGPAGAGESKCPLMVKVLDAVRGSPAVDVAVKVFKKTSEGSWEPFASGKTAESGELHGLTTDEKFVEGVYRVELDTKSYWKTLGISPFHEFADVVFTANDSGHRHYTIAALLSPYSYSTTAVVSNPQN

SEQ ID NO: 7 - DNA, 1237 bp, Mus musculus
ctaatctccctaggcaaggttcatatttgtgtaggttacttattctccttttgttgactaagtcaataatcagaatcagcaggtttggagtcagcttggcagggatcagcagcctgggttggaaggagggggtataaaagccccttcaccaggagaagccgtcacacagatccacaagctcctgacaggatggcttcccttcgactcttcctcctttgcctcgctggactggtatttgtgtctgaagctggccccgcgggtgctggagaatccaaatgtcctctgatggtcaaagtcctggatgctgtccgaggcagccctgctgtagacgtggctgtaaaagtgttcaaaaagacctctgagggatcctgggagccctttgcctctgggaagaccgcggagtctggagagctgcacgggctcaccacagatgagaagtttgtagaaggagtgtacagagtagaactggacaccaaatcgtactggaagacacttggcatttccccgttccatgaattcgcggatgtggttttcacagccaacgactctggccatcgccactacaccatcgcagccctgctcagcccatactcctacagcaccacggctgtcgtcagcaacccccagaattgagagactcagcccaggaggaccaggatcttgccaaagcagtagcatcccatttgtaccaaaacagtgttcttgctctataaaccgtgttagcagctcaggaagatgccgtgaagcattcttattaaaccacctgctatttcattcaaactgtgtttcttttttatttcctcatttttctcccctgctcctaaaacccaaaatcttctaaagaattctagaaggtatgcgatcaaactttttaaagaaagaaaatactttttgactcatggtttaaaggcatcctttccatcttggggaggtcatgggtgctcctggcaacttgcttgaggaagataggtcagaaagcagagtggaccaaccgttcaatgttttacaagcaaaacatacactaagcatggtctgtagctattaaaagcacacaatctgaagggctgtagatgcacagtagtgttttcccagagcatgttcaaaagccctgggttcaatcacaatactgaaaagtaggccaaaaaacattctgaaaatgaaatatttgggtttttttttataacctttagtgactaaataaagacaaatctaagagactaaaaaaaaaaaaaaaaaa

SEQ ID NO: 8 - RNA, 82 nt, Artificial Sequence
  Synthetic
guuggaaccauucaaaacagcauagcaaguuaaaauaaggcuaguccguuaucaacuugaaaaaguggcaccgagucggugc

SEQ ID NO: 9 - RNA, 76 nt, Artificial Sequence
  Synthetic
guuuuagagcuagaaauagcaaguuaaaauaaggcuaguccguuaucaacuugaaaaaguggcaccgagucggugc

SEQ ID NO: 10 - RNA, 86 nt, Artificial Sequence
  Synthetic
guuuaagagcuaugcuggaaacagcauagcaaguuuaaauaaggcuaguccguuaucaacuugaaaaaguggcaccgagucggugc

SEQ ID NO: 11 - DNA, 23 bp, Artificial Sequence
  Synthetic
  misc_feature (2)..(21): n = A, T, C, or G
gnnnnnnnnnnnnnnnnnnnngg

SEQ ID NO: 12 - DNA, 23 bp, Artificial Sequence
  Synthetic
  misc_feature (1)..(21): n = A, T, C, or G
nnnnnnnnnnnnnnnnnnnnngg

SEQ ID NO: 13 - DNA, 25 bp, Artificial Sequence
  Synthetic
  misc_feature (3)..(23): n = A, T, C, or G
ggnnnnnnnnnnnnnnnnnnnnngg

SEQ ID NO: 14 - DNA, 12208 bp, Artificial Sequence
  Synthetic
  misc_feature (1)..(97): Mouse Sequence
  misc_feature (98)..(7298): Human Sequence
  misc_feature (7299)..(12108): SDC Neo Cassette
  misc_feature (12109)..(12208): Mouse Sequence
agcttggcagggatcagcagcctgggttggaaggagggggtataaaagccccttcaccaggagaagccgtcacacagatccacaagctcctgacaggatggcttctcatcgtctgctcctcctctgccttgctggactggtatttgtgtctgaggctggccctacggtgagtgtttctgtgacatcccattcctacatttaagattcacgctaaatgaagtagaagtgactccttccagctttgccaaccagcttttattactagggcaagggtacccagcatctatttttaatataattaattcaaacttcaaaaagaatgaagttccactgagcttactgagctgggacttgaactctgagcattctacctcattgctttggtgcattaggtttgtaatatctggtacctctgtttcctcagatagatgatagaaataaagatatgatattaaggaagctgttaatactgaattttcagaaaagtatccctccataaaatgtatttgggggacaaactgcaggagattatattctggccctatagttattcaaaacgtatttattgattaatctttaaaaggcttagtgaacaatattctagtcagatatctaattcttaaatcctctagaagaattaactaatactataaaatgggtctggatgtagttctgacattattttataacaactggtaagagggagtgactatagcaacaactaaaatgatctcaggaaaacctgtttggccctatgtatggtacattacatcttttcagtaattccactcaaatggagacttttaacaaagcaactgttctcaggggacctattttctcccttaaaattcattatacacatccctggttgatagcagtgtgtctggaggcagaaaccattcttgctttggaaacaattacgtctgtgttatactgagtagggaagctcattaattgtcgacacttacgttcctgataatgggatcagtgtgtaattcttgtttcgctccagatttctaataccacaaagaataaatcctttcactctgatcaattttgttaacttctcacgtgtcttctctacacccagggcaccggtgaatccaagtgtcctctgatggtcaaagttctagatgctgtccgaggcagtcctgccatcaatgtggccgtgcatgtgttcagaaaggctgctgatgacacctgggagccatttgcctctgggtaagttgccaaagaaccctcccacaggacttggttttatcttcccgtttgcccctcacttggtagagagaggctcacatcatctgctaaagaatttacaagtagattgaaaaacgtaggcagaggtcaagtatgccctctgaaggatgccctctttttgttttgcttagctaggaagtgaccaggaacctgagcatcatttaggggcagacagtagagaaaagaaggaatcagaactcctctcctctagctgtggtttgcaacccttttgggtcacagaacactttatgtaggtgatgaaaagtaaacattctatgcccagaaaaaatgcacagatacacacacatacaaaatcatatatgtgattttaggagtttcacagattccctggtgtccctgggtaacaccaaagctaagtgtccttgtcttagaattttaggaaaaggtataatgtgtattaacccattaacaaaaggaaaggaattcagaaatattattaaccaggcatctgtctgtagttaatatggatcacccaaaacccaaggcttttgcctaatgaacactttggggcacctactgtgtgcaaggctgggggctgtcaagctcagttaaaaaaaaaaagatagaagagatggatccatgaggcaaagtacagccccaggctaatcccacgatcacccgacttcatgtccaagagtggcttctcaccttcattagccagttcacaattttcatggagtttttctacctgcactagcaaaaacttcaaggaaaatacatattaataaatctaagcaaagtgaccagaagacagagcaatcaggagaccctttgcatccagcagaagaggaactgctaagtatttacatctccacagagaagaatttctgttgggttttaattgaaccccaagaaccacatgattcttcaaccattattgggaagatcattttcttaggtctggttttaactggctttttatttgggaattcatttatgtttatataaaatgccaagcataacatgaaaagtggttacaggactattctaagggagagacagaatggacaccaaaaatattccaatgttcttgtgaatcttttccttgcaccaggacaaaaaaaaaaagaagtgaaaagaagaaaggaggaggggcataatcagagtcagtaaagacaactgctatttttatctatcgtagctgttgcagtcaaatgggaagcaatttccaacattcaactatggagctggtacttacatggaaatagaagttgcctagtgtttgttgctggcaaagagttatcagagaggttaaatatataaaagggaaaagagtcagatacaggttcttcttcctactttaggttttccactgtgtgtgcaaatgatactccctggtggtgtgcagatgcctcaaagctatcctcacaccacaagggagaggagcgagatcctgctgtcctggagaagtgcagagttagaacagctgtggccacttgcatccaatcatcaatcttgaatcacagggactctttcttaagtaaacattatacctggccgggcacggtggctcacgcctgtaatcccagcactttgggatgccaaagtgggcatatcatctgaggtcaggagttcaagaccagcctggccaacatggcaaaactccgtctttatgaaaaatacaaaaattagccaggcatggtggcaggcgcctgtaatcccagctaattgggaggctgaggctggagaatcccttgaatctaggaggcagaggttgcagtgagctgagatcgtgccattgcactccagcctgggtgacaagagtaaaactctgtctcaaaaaaaaaaaattatacctacattctcttcttatcagagaaaaaaatctacagtgagcttttcaaaaagtttttacaaactttttgccatttaatttcagttaggagttttccctacttctgacttagttgaggggaaatgttcataacatgtttataacatgtttatgtgtgttagttggtgggggtgtattactttgccatgccatttgtttcctccatgcgtaacttaatccagactttcacaccttataggaaaaccagtgagtctggagagctgcatgggctcacaactgaggaggaatttgtagaagggatatacaaagtggaaatagacaccaaatcttactggaaggcacttggcatctccccattccatgagcatgcagaggtgagtatacagaccttcgagggttgttttggttttggtttttgcttttggcattccaggaaatgcacagttttactcagtgtaccacagaaatgtcctaaggaaggtgatgaatgaccaaaggttccctttcctattatacaagaaaaaattcacaacactctgagaagcaaatttctttttgactttgatgaaaatccacttagtaacatgacttgaacttacatgaaactactcatagtctattcattccactttatatgaatattgatgtatctgctgttgaaataatagtttatgaggcagccctccagaccccacgtagagtgtatgtaacaagagatgcaccattttatttctcgaaaacccgtaacattcttcattccaaaacacatctggcttctcggaggtctggacaagtgattcttggcaacacatacctatagagacaataaaatcaaagtaataatggcaacacaatagataacatttaccaagcatacaccatgtggcagacacaattataagtgttttccatatttaacctacttaatcctcaggaataagccactgaggtcagtcctattattatccccatcttatagatgaagaaaatgaggcaccaggaagtcaaataacttgtcaaaggtcacaagactaggaaatacacaagtagaaatgtttacaattaaggcccaggctgggtttgccctcagttctgctatgcctcgcattatgccccaggaaactttttcccttgtgaaagccaagcttaaaaaaagaaaagccacatttgtaacgtgctctgttcccctgcctatggtgaggatcttcaaacagttatacatggacccagtccccctgccttctccttaatttcttaagtcatttgaaacagatggctgtcatggaaatagaatccagacatgttggtcagagttaaagatcaactaattccatcaaaaatagctcggcatgaaagggaactattctctggcttagtcatggatgagactttcaattgctataaagtggttcctttattagacaatgttaccagggaaacaacaggggtttgtttgacttctggggcccacaagtcaacaagagagccccatctaccaaggagcatgtccctgactacccctcagccagcagcaagacatggaccccagtcagggcaggagcagggtttcggcggcgcccagcacaagacattgcccctagagtctcagcccctaccctcgagtaatagatctgcctacctgagactgttgtttgcccaagagctgggtctcagcctgatgggaaccatataaaaaggttcactgacatactgcccacatgttgttctctttcattagatcttagcttccttgtctgctcttcattcttgcagtattcattcaacaaacattaaaaaaaaaaaaaagcattctatgtgtggaacactctgctagatgctgtggatttagaaatgaaaatacatcccgacccttggaatggaagggaaaggactgaagtaagacagattaagcaggaccgtcagcccagcttgaagcccagataaatacggagaacaagagagagcgagtagtgagagatgagtcccaatgcctcactttggtgacgggtgcgtggtgggcttcatgcagcttcttctgataaatgcctccttcagaactggtcaactctaccttggccagtgacccaggtggtcatagtagatttaccaagggaaaatggaaacttttattaggagctcttaggcctcttcacttcatggatttttttttcctttttttttgagatggagttttgccctgtcacccaggctggaatgcagtggtgcaatctcagctcactgcaacctccgcctcccaggttcaagcaattctcctgcctcagcctcccgagtagctgggactacaggtgtgcgccaccacaccaggctaatttttgtattttttgtaaagacaggttttcaccacgttggccaggctggtctgaactccagacctcaggtgattcacctgtctcagcctcccaaagtgctgggattacaggtgtgagccaccgtgcccggctacttcatggatttttgattacagattatgcctcttacaatttttaagaagaatcaagtgggctgaaggtcaatgtcaccataagacaaaagacatttttattagttgattctagggaattggccttaaggggagccctttcttcctaagagattcttaggtgattctcacttcctcttgccccagtattatttttgtttttggtatggctcactcagatccttttttcctcctatccctaagtaatccgggtttctttttcccatatttagaacaaaatgtatttatgcagagtgtgtccaaacctcaacccaaggcctgtatacaaaataaatcaaattaaacacatctttactgtcttctacctctttcctgacctcaatatatcccaacttgcctcactctgagaaccaaggctgtcccagcacctgagtcgcagatattctactgatttgacagaactgtgtgactatctggaacagcattttgatccacaatttgcccagttacaaagcttaaatgagctctagtgcatgcatatatatttcaaaattccaccatgatcttccacactctgtattgtaaatagagccctgtaatgcttttacttcgtatttcattgcttgttatacataaaaatatacttttcttcttcatgttagaaaatgcaaagaataggagggtgggggaatctctgggcttggagacaggagacttgccttcctactatggttccatcagaatgtagactgggacaatacaataattcaagtctggtttgctcatctgtaaattgggaagaatgtttccagctccagaatgctaaatctctaagtctgtggttggcagccactattgcagcagctcttcaatgactcaatgcagttttgcattctccctaccttttttttctaaaaccaataaaatagatacagcctttaggctttctgggatttcccttagtcaagctagggtcatcctgactttcggcgtgaatttgcaaaacaagacctgactctgtactcctgctctaaggactgtgcatggttccaaaggcttagcttgccagcatatttgagctttttccttctgttcaaactgttccaaaatataaaagaataaaattaattaagttggcactggacttccggtggtcagtcatgtgtgtcatctgtcacgtttttcgggctctggtggaaatggatctgtctgtcttctctcataggtggtattcacagccaacgactccggcccccgccgctacaccattgccgccctgctgagcccctactcctattccaccacggctgtcgtcaccaatcccaaggaatgagggacttctcctccagtggacctgaaggacgagggatgggatttcatgtaaccaagagtattccatttttactaaagcagtgttttcacctcatatgctatgttagaagtccaggcagagacaataaaacattcctgtgaaaggcacttttcattccactttaacttgattttttaaattcccttattgtcccttccaaaaaaaagagaatcaaaattttacaaagaatcaaaggaattctagaaagtatctgggcagaacgctaggagagatccaaatttccattgtcttgcaagcaaagcacgtattaaatatgatctgcagccattaaaaagacacattctgtaaatgagagagccttattttcctgtaaccttcagcaaatagcaaaagacacattccaagggcccacttctttactgtgggcactcgagataacttcgtataatgtatgctatacgaagttatatgcatgccagtagcagcacccacgtccaccttctgtctagtaatgtccaacacctccctcagtccaaacactgctctgcatccatgtggctcccatttatacctgaagcacttgatggggcctcaatgttttactagagcccacccccctgcaactctgagaccctctggatttgtctgtcagtgcctcactggggcgttggataatttcttaaaaggtcaagttccctcagcagcattctctgagcagtctgaagatgtgtgcttttcacagttcaaatccatgtggctgtttcacccacctgcctggccttgggttatctatcaggacctagcctagaagcaggtgtgtggcacttaacacctaagctgagtgactaactgaacactcaagtggatgccatctttgtcacttcttgactgtgacacaagcaactcctgatgccaaagccctgcccacccctctcatgcccatatttggacatggtacaggtcctcactggccatggtctgtgaggtcctggtcctctttgacttcataattcctaggggccactagtatctataagaggaagagggtgctggctcccaggccacagcccacaaaattccacctgctcacaggttggctggctcgacccaggtggtgtcccctgctctgagccagctcccggccaagccagcaccatgggaacccccaagaagaagaggaaggtgcgtaccgatttaaattccaatttactgaccgtacaccaaaatttgcctgcattaccggtcgatgcaacgagtgatgaggttcgcaagaacctgatggacatgttcagggatcgccaggcgttttctgagcatacctggaaaatgcttctgtccgtttgccggtcgtgggcggcatggtgcaagttgaataaccggaaatggtttcccgcagaacctgaagatgttcgcgattatcttctatatcttcaggcgcgcggtctggcagtaaaaactatccagcaacatttgggccagctaaacatgcttcatcgtcggtccgggctgccacgaccaagtgacagcaatgctgtttcactggttatgcggcggatccgaaaagaaaacgttgatgccggtgaacgtgcaaaacaggtaaatataaaatttttaagtgtataatgatgttaaactactgattctaattgtttgtgtattttaggctctagcgttcgaacgcactgatttcgaccaggttcgttcactcatggaaaatagcgatcgctgccaggatatacgtaatctggcatttctggggattgcttataacaccctgttacgtatagccgaaattgccaggatcagggttaaagatatctcacgtactgacggtgggagaatgttaatccatattggcagaacgaaaacgctggttagcaccgcaggtgtagagaaggcacttagcctgggggtaactaaactggtcgagcgatggatttccgtctctggtgtagctgatgatccgaataactacctgttttgccgggtcagaaaaaatggtgttgccgcgccatctgccaccagccagctatcaactcgcgccctggaagggatttttgaagcaactcatcgattgatttacggcgctaaggatgactctggtcagagatacctggcctggtctggacacagtgcccgtgtcggagccgcgcgagatatggcccgcgctggagtttcaataccggagatcatgcaagctggtggctggaccaatgtaaatattgtcatgaactatatccgtaacctggatagtgaaacaggggcaatggtgcgcctgctggaagatggcgattaggcggccggccgctaatcagccataccacatttgtagaggttttacttgctttaaaaaacctcccacacctccccctgaacctgaaacataaaatgaatgcaattgttgttgttaacttgtttattgcagcttataatggttacaaataaagcaatagcatcacaaatttcacaaataaagcatttttttcactgcattctagttgtggtttgtccaaactcatcaatgtatcttatcatgtctggatcccccggctagagtttaaacactagaactagtggatcccccgggatcatggcctccgcgccgggttttggcgcctcccgcgggcgcccccctcctcacggcgagcgctgccacgtcagacgaagggcgcagcgagcgtcctgatccttccgcccggacgctcaggacagcggcccgctgctcataagactcggccttagaaccccagtatcagcagaaggacattttaggacgggacttgggtgactctagggcactggttttctttccagagagcggaacaggcgaggaaaagtagtcccttctcggcgattctgcggagggatctccgtggggcggtgaacgccgatgattatataaggacgcgccgggtgtggcacagctagttccgtcgcagccgggatttgggtcgcggttcttgtttgtggatcgctgtgatcgtcacttggtgagtagcgggctgctgggctggccggggctttcgtggccgccgggccgctcggtgggacggaagcgtgtggagagaccgccaagggctgtagtctgggtccgcgagcaaggttgccctgaactgggggttggggggagcgcagcaaaatggcggctgttcccgagtcttgaatggaagacgcttgtgaggcgggctgtgaggtcgttgaaacaaggtggggggcatggtgggcggcaagaacccaaggtcttgaggccttcgctaatgcgggaaagctcttattcgggtgagatgggctggggcaccatctggggaccctgacgtgaagtttgtcactgactggagaactcggtttgtcgtctgttgcgggggcggcagttatggcggtgccgttgggcagtgcacccgtacctttgggagcgcgcgccctcgtcgtgtcgtgacgtcacccgttctgttggcttataatgcagggtggggccacctgccggtaggtgtgcggtaggcttttctccgtcgcaggacgcagggttcgggcctagggtaggctctcctgaatcgacaggcgccggacctctggtgaggggagggataagtgaggcgtcagtttctttggtcggttttatgtacctatcttcttaagtagctgaagctccggttttgaactatgcgctcggggttggcgagtgtgttttgtgaagttttttaggcaccttttgaaatgtaatcatttgggtcaatatgtaattttcagtgttagactagtaaattgtccgctaaattctggccgtttttggcttttttgttagacgtgttgacaattaatcatcggcatagtatatcggcatagtataatacgacaaggtgaggaactaaaccatgggatcggccattgaacaagatggattgcacgcaggttctccggccgcttgggtggagaggctattcggctatgactgggcacaacagacaatcggctgctctgatgccgccgtgttccggctgtcagcgcaggggcgcccggttctttttgtcaagaccgacctgtccggtgccctgaatgaactgcaggacgaggcagcgcggctatcgtggctggccacgacgggcgttccttgcgcagctgtgctcgacgttgtcactgaagcgggaagggactggctgctattgggcgaagtgccggggcaggatctcctgtcatctcaccttgctcctgccgagaaagtatccatcatggctgatgcaatgcggcggctgcatacgcttgatccggctacctgcccattcgaccaccaagcgaaacatcgcatcgagcgagcacgtactcggatggaagccggtcttgtcgatcaggatgatctggacgaagagcatcaggggctcgcgccagccgaactgttcgccaggctcaaggcgcgcatgcccgacggcgatgatctcgtcgtgacccatggcgatgcctgcttgccgaatatcatggtggaaaatggccgcttttctggattcatcgactgtggccggctgggtgtggcggaccgctatcaggacatagcgttggctacccgtgatattgctgaagagcttggcggcgaatgggctgaccgcttcctcgtgctttacggtatcgccgctcccgattcgcagcgcatcgccttctatcgccttcttgacgagttcttctgaggggatccgctgtaagtctgcagaaattgatgatctattaaacaataaagatgtccactaaaatggaagtttttcctgtcatactttgttaagaagggtgagaacagagtacctacattttgaatggaaggattggagctacgggggtgggggtggggtgggattagataaatgcctgctctttactgaaggctctttactattgctttatgataatgtttcatagttggatatcataatttaaacaagcaaaaccaaattaagggccagctcattcctcccactcatgatctatagatctatagatctctcgtgggatcattgtttttctcttgattcccactttgtggttctaagtactgtggtttccaaatgtgtcagtttcatagcctgaagaacgagatcagcagcctctgttccacatacacttcattctcagtattgttttgccaagttctaattccatcagacctcgacctgcagcccctagataacttcgtataatgtatgctatacgaagttatgctaggtaactataacggtcctaaggtagcgagctagcgagactcagcccaggaggaccaggatcttgccaaagcagtagcatcccatttgtaccaaaacagtgttcttgctctataaaccgtgttagcagctcagga

SEQ ID NO: 15 - DNA, 7476 bp, Artificial Sequence
  Synthetic
  misc_feature (1)..(97): Mouse Sequence
  misc_feature (98)..(7298): Human Sequence
  misc_feature (7299)..(7376): Cassette LoxP Scar
  misc_feature (7377)..(7476): Mouse Sequence
agcttggcagggatcagcagcctgggttggaaggagggggtataaaagccccttcaccaggagaagccgtcacacagatccacaagctcctgacaggatggcttctcatcgtctgctcctcctctgccttgctggactggtatttgtgtctgaggctggccctacggtgagtgtttctgtgacatcccattcctacatttaagattcacgctaaatgaagtagaagtgactccttccagctttgccaaccagcttttattactagggcaagggtacccagcatctatttttaatataattaattcaaacttcaaaaagaatgaagttccactgagcttactgagctgggacttgaactctgagcattctacctcattgctttggtgcattaggtttgtaatatctggtacctctgtttcctcagatagatgatagaaataaagatatgatattaaggaagctgttaatactgaattttcagaaaagtatccctccataaaatgtatttgggggacaaactgcaggagattatattctggccctatagttattcaaaacgtatttattgattaatctttaaaaggcttagtgaacaatattctagtcagatatctaattcttaaatcctctagaagaattaactaatactataaaatgggtctggatgtagttctgacattattttataacaactggtaagagggagtgactatagcaacaactaaaatgatctcaggaaaacctgtttggccctatgtatggtacattacatcttttcagtaattccactcaaatggagacttttaacaaagcaactgttctcaggggacctattttctcccttaaaattcattatacacatccctggttgatagcagtgtgtctggaggcagaaaccattcttgctttggaaacaattacgtctgtgttatactgagtagggaagctcattaattgtcgacacttacgttcctgataatgggatcagtgtgtaattcttgtttcgctccagatttctaataccacaaagaataaatcctttcactctgatcaattttgttaacttctcacgtgtcttctctacacccagggcaccggtgaatccaagtgtcctctgatggtcaaagttctagatgctgtccgaggcagtcctgccatcaatgtggccgtgcatgtgttcagaaaggctgctgatgacacctgggagccatttgcctctgggtaagttgccaaagaaccctcccacaggacttggttttatcttcccgtttgcccctcacttggtagagagaggctcacatcatctgctaaagaatttacaagtagattgaaaaacgtaggcagaggtcaagtatgccctctgaaggatgccctctttttgttttgcttagctaggaagtgaccaggaacctgagcatcatttaggggcagacagtagagaaaagaaggaatcagaactcctctcctctagctgtggtttgcaacccttttgggtcacagaacactttatgtaggtgatgaaaagtaaacattctatgcccagaaaaaatgcacagatacacacacatacaaaatcatatatgtgattttaggagtttcacagattccctggtgtccctgggtaacaccaaagctaagtgtccttgtcttagaattttaggaaaaggtataatgtgtattaacccattaacaaaaggaaaggaattcagaaatattattaaccaggcatctgtctgtagttaatatggatcacccaaaacccaaggcttttgcctaatgaacactttggggcacctactgtgtgcaaggctgggggctgtcaagctcagttaaaaaaaaaaagatagaagagatggatccatgaggcaaagtacagccccaggctaatcccacgatcacccgacttcatgtccaagagtggcttctcaccttcattagccagttcacaattttcatggagtttttctacctgcactagcaaaaacttcaaggaaaatacatattaataaatctaagcaaagtgaccagaagacagagcaatcaggagaccctttgcatccagcagaagaggaactgctaagtatttacatctccacagagaagaatttctgttgggttttaattgaaccccaagaaccacatgattcttcaaccattattgggaagatcattttcttaggtctggttttaactggctttttatttgggaattcatttatgtttatataaaatgccaagcataacatgaaaagtggttacaggactattctaagggagagacagaatggacaccaaaaatattccaatgttcttgtgaatcttttccttgcaccaggacaaaaaaaaaaagaagtgaaaagaagaaaggaggaggggcataatcagagtcagtaaagacaactgctatttttatctatcgtagctgttgcagtcaaatgggaagcaatttccaacattcaactatggagctggtacttacatggaaatagaagttgcctagtgtttgttgctggcaaagagttatcagagaggttaaatatataaaagggaaaagagtcagatacaggttcttcttcctactttaggttttccactgtgtgtgcaaatgatactccctggtggtgtgcagatgcctcaaagctatcctcacaccacaagggagaggagcgagatcctgctgtcctggagaagtgcagagttagaacagctgtggccacttgcatccaatcatcaatcttgaatcacagggactctttcttaagtaaacattatacctggccgggcacggtggctcacgcctgtaatcccagcactttgggatgccaaagtgggcatatcatctgaggtcaggagttcaagaccagcctggccaacatggcaaaactccgtctttatgaaaaatacaaaaattagccaggcatggtggcaggcgcctgtaatcccagctaattgggaggctgaggctggagaatcccttgaatctaggaggcagaggttgcagtgagctgagatcgtgccattgcactccagcctgggtgacaagagtaaaactctgtctcaaaaaaaaaaaattatacctacattctcttcttatcagagaaaaaaatctacagtgagcttttcaaaaagtttttacaaactttttgccatttaatttcagttaggagttttccctacttctgacttagttgaggggaaatgttcataacatgtttataacatgtttatgtgtgttagttggtgggggtgtattactttgccatgccatttgtttcctccatgcgtaacttaatccagactttcacaccttataggaaaaccagtgagtctggagagctgcatgggctcacaactgaggaggaatttgtagaagggatatacaaagtggaaatagacaccaaatcttactggaaggcacttggcatctccccattccatgagcatgcagaggtgagtatacagaccttcgagggttgttttggttttggtttttgcttttggcattccaggaaatgcacagttttactcagtgtaccacagaaatgtcctaaggaaggtgatgaatgaccaaaggttccctttcctattatacaagaaaaaattcacaacactctgagaagcaaatttctttttgactttgatgaaaatccacttagtaacatgacttgaacttacatgaaactactcatagtctattcattccactttatatgaatattgatgtatctgctgttgaaataatagtttatgaggcagccctccagaccccacgtagagtgtatgtaacaagagatgcaccattttatttctcgaaaacccgtaacattcttcattccaaaacacatctggcttctcggaggtctggacaagtgattcttggcaacacatacctatagagacaataaaatcaaagtaataatggcaacacaatagataacatttaccaagcatacaccatgtggcagacacaattataagtgttttccatatttaacctacttaatcctcaggaataagccactgaggtcagtcctattattatccccatcttatagatgaagaaaatgaggcaccaggaagtcaaataacttgtcaaaggtcacaagactaggaaatacacaagtagaaatgtttacaattaaggcccaggctgggtttgccctcagttctgctatgcctcgcattatgccccaggaaactttttcccttgtgaaagccaagcttaaaaaaagaaaagccacatttgtaacgtgctctgttcccctgcctatggtgaggatcttcaaacagttatacatggacccagtccccctgccttctccttaatttcttaagtcatttgaaacagatggctgtcatggaaatagaatccagacatgttggtcagagttaaagatcaactaattccatcaaaaatagctcggcatgaaagggaactattctctggcttagtcatggatgagactttcaattgctataaagtggttcctttattagacaatgttaccagggaaacaacaggggtttgtttgacttctggggcccacaagtcaacaagagagccccatctaccaaggagcatgtccctgactacccctcagccagcagcaagacatggaccccagtcagggcaggagcagggtttcggcggcgcccagcacaagacattgcccctagagtctcagcccctaccctcgagtaatagatctgcctacctgagactgttgtttgcccaagagctgggtctcagcctgatgggaaccatataaaaaggttcactgacatactgcccacatgttgttctctttcattagatcttagcttccttgtctgctcttcattcttgcagtattcattcaacaaacattaaaaaaaaaaaaaagcattctatgtgtggaacactctgctagatgctgtggatttagaaatgaaaatacatcccgacccttggaatggaagggaaaggactgaagtaagacagattaagcaggaccgtcagcccagcttgaagcccagataaatacggagaacaagagagagcgagtagtgagagatgagtcccaatgcctcactttggtgacgggtgcgtggtgggcttcatgcagcttcttctgataaatgcctccttcagaactggtcaactctaccttggccagtgacccaggtggtcatagtagatttaccaagggaaaatggaaacttttattaggagctcttaggcctcttcacttcatggatttttttttcctttttttttgagatggagttttgccctgtcacccaggctggaatgcagtggtgcaatctcagctcactgcaacctccgcctcccaggttcaagcaattctcctgcctcagcctcccgagtagctgggactacaggtgtgcgccaccacaccaggctaatttttgtattttttgtaaagacaggttttcaccacgttggccaggctggtctgaactccagacctcaggtgattcacctgtctcagcctcccaaagtgctgggattacaggtgtgagccaccgtgcccggctacttcatggatttttgattacagattatgcctcttacaatttttaagaagaatcaagtgggctgaaggtcaatgtcaccataagacaaaagacatttttattagttgattctagggaattggccttaaggggagccctttcttcctaagagattcttaggtgattctcacttcctcttgccccagtattatttttgtttttggtatggctcactcagatccttttttcctcctatccctaagtaatccgggtttctttttcccatatttagaacaaaatgtatttatgcagagtgtgtccaaacctcaacccaaggcctgtatacaaaataaatcaaattaaacacatctttactgtcttctacctctttcctgacctcaatatatcccaacttgcctcactctgagaaccaaggctgtcccagcacctgagtcgcagatattctactgatttgacagaactgtgtgactatctggaacagcattttgatccacaatttgcccagttacaaagcttaaatgagctctagtgcatgcatatatatttcaaaattccaccatgatcttccacactctgtattgtaaatagagccctgtaatgcttttacttcgtatttcattgcttgttatacataaaaatatacttttcttcttcatgttagaaaatgcaaagaataggagggtgggggaatctctgggcttggagacaggagacttgccttcctactatggttccatcagaatgtagactgggacaatacaataattcaagtctggtttgctcatctgtaaattgggaagaatgtttccagctccagaatgctaaatctctaagtctgtggttggcagccactattgcagcagctcttcaatgactcaatgcagttttgcattctccctaccttttttttctaaaaccaataaaatagatacagcctttaggctttctgggatttcccttagtcaagctagggtcatcctgactttcggcgtgaatttgcaaaacaagacctgactctgtactcctgctctaaggactgtgcatggttccaaaggcttagcttgccagcatatttgagctttttccttctgttcaaactgttccaaaatataaaagaataaaattaattaagttggcactggacttccggtggtcagtcatgtgtgtcatctgtcacgtttttcgggctctggtggaaatggatctgtctgtcttctctcataggtggtattcacagccaacgactccggcccccgccgctacaccattgccgccctgctgagcccctactcctattccaccacggctgtcgtcaccaatcccaaggaatgagggacttctcctccagtggacctgaaggacgagggatgggatttcatgtaaccaagagtattccatttttactaaagcagtgttttcacctcatatgctatgttagaagtccaggcagagacaataaaacattcctgtgaaaggcacttttcattccactttaacttgattttttaaattcccttattgtcccttccaaaaaaaagagaatcaaaattttacaaagaatcaaaggaattctagaaagtatctgggcagaacgctaggagagatccaaatttccattgtcttgcaagcaaagcacgtattaaatatgatctgcagccattaaaaagacacattctgtaaatgagagagccttattttcctgtaaccttcagcaaatagcaaaagacacattccaagggcccacttctttactgtgggcactcgagataacttcgtataatgtatgctatacgaagttatgctaggtaactataacggtcctaaggtagcgagctagcgagactcagcccaggaggaccaggatcttgccaaagcagtagcatcccatttgtaccaaaacagtgttcttgctctataaaccgtgttagcagctcagga

SEQ ID NO: 16 - DNA, 11218 bp, Artificial Sequence
  Synthetic
  misc_feature (1)..(100): Mouse Sequence
  misc_feature (101)..(6308): Human Sequence
  misc_feature (6309)..(11118): SDC Neo Cassette
  misc_feature (11119)..(11218): Mouse Sequence
atgtacttttggttttgttccagagtctatcaccggaaagaacaagccggtttactctgacccatttcactgacatttctcttgtctcctctgtgcccagggcaccggtgaatccaagtgtcctctgatggtcaaagttctagatgctgtccgaggcagtcctgccatcaatgtggccgtgcatgtgttcagaaaggctgctgatgacacctgggagccatttgcctctgggtaagttgccaaagaaccctcccacaggacttggttttatcttcccgtttgcccctcacttggtagagagaggctcacatcatctgctaaagaatttacaagtagattgaaaaacgtaggcagaggtcaagtatgccctctgaaggatgccctctttttgttttgcttagctaggaagtgaccaggaacctgagcatcatttaggggcagacagtagagaaaagaaggaatcagaactcctctcctctagctgtggtttgcaacccttttgggtcacagaacactttatgtaggtgatgaaaagtaaacattctatgcccagaaaaaatgcacagatacacacacatacaaaatcatatatgtgattttaggagtttcacagattccctggtgtccctgggtaacaccaaagctaagtgtccttgtcttagaattttaggaaaaggtataatgtgtattaacccattaacaaaaggaaaggaattcagaaatattattaaccaggcatctgtctgtagttaatatggatcacccaaaacccaaggcttttgcctaatgaacactttggggcacctactgtgtgcaaggctgggggctgtcaagctcagttaaaaaaaaaaagatagaagagatggatccatgaggcaaagtacagccccaggctaatcccacgatcacccgacttcatgtccaagagtggcttctcaccttcattagccagttcacaattttcatggagtttttctacctgcactagcaaaaacttcaaggaaaatacatattaataaatctaagcaaagtgaccagaagacagagcaatcaggagaccctttgcatccagcagaagaggaactgctaagtatttacatctccacagagaagaatttctgttgggttttaattgaaccccaagaaccacatgattcttcaaccattattgggaagatcattttcttaggtctggttttaactggctttttatttgggaattcatttatgtttatataaaatgccaagcataacatgaaaagtggttacaggactattctaagggagagacagaatggacaccaaaaatattccaatgttcttgtgaatcttttccttgcaccaggacaaaaaaaaaaagaagtgaaaagaagaaaggaggaggggcataatcagagtcagtaaagacaactgctatttttatctatcgtagctgttgcagtcaaatgggaagcaatttccaacattcaactatggagctggtacttacatggaaatagaagttgcctagtgtttgttgctggcaaagagttatcagagaggttaaatatataaaagggaaaagagtcagatacaggttcttcttcctactttaggttttccactgtgtgtgcaaatgatactccctggtggtgtgcagatgcctcaaagctatcctcacaccacaagggagaggagcgagatcctgctgtcctggagaagtgcagagttagaacagctgtggccacttgcatccaatcatcaatcttgaatcacagggactctttcttaagtaaacattatacctggccgggcacggtggctcacgcctgtaatcccagcactttgggatgccaaagtgggcatatcatctgaggtcaggagttcaagaccagcctggccaacatggcaaaactccgtctttatgaaaaatacaaaaattagccaggcatggtggcaggcgcctgtaatcccagctaattgggaggctgaggctggagaatcccttgaatctaggaggcagaggttgcagtgagctgagatcgtgccattgcactccagcctgggtgacaagagtaaaactctgtctcaaaaaaaaaaaattatacctacattctcttcttatcagagaaaaaaatctacagtgagcttttcaaaaagtttttacaaactttttgccatttaatttcagttaggagttttccctacttctgacttagttgaggggaaatgttcataacatgtttataacatgtttatgtgtgttagttggtgggggtgtattactttgccatgccatttgtttcctccatgcgtaacttaatccagactttcacaccttataggaaaaccagtgagtctggagagctgcatgggctcacaactgaggaggaatttgtagaagggatatacaaagtggaaatagacaccaaatcttactggaaggcacttggcatctccccattccatgagcatgcagaggtgagtatacagaccttcgagggttgttttggttttggtttttgcttttggcattccaggaaatgcacagttttactcagtgtaccacagaaatgtcctaaggaaggtgatgaatgaccaaaggttccctttcctattatacaagaaaaaattcacaacactctgagaagcaaatttctttttgactttgatgaaaatccacttagtaacatgacttgaacttacatgaaactactcatagtctattcattccactttatatgaatattgatgtatctgctgttgaaataatagtttatgaggcagccctccagaccccacgtagagtgtatgtaacaagagatgcaccattttatttctcgaaaacccgtaacattcttcattccaaaacacatctggcttctcggaggtctggacaagtgattcttggcaacacatacctatagagacaataaaatcaaagtaataatggcaacacaatagataacatttaccaagcatacaccatgtggcagacacaattataagtgttttccatatttaacctacttaatcctcaggaataagccactgaggtcagtcctattattatccccatcttatagatgaagaaaatgaggcaccaggaagtcaaataacttgtcaaaggtcacaagactaggaaatacacaagtagaaatgtttacaattaaggcccaggctgggtttgccctcagttctgctatgcctcgcattatgccccaggaaactttttcccttgtgaaagccaagcttaaaaaaagaaaagccacatttgtaacgtgctctgttcccctgcctatggtgaggatcttcaaacagttatacatggacccagtccccctgccttctccttaatttcttaagtcatttgaaacagatggctgtcatggaaatagaatccagacatgttggtcagagttaaagatcaactaattccatcaaaaatagctcggcatgaaagggaactattctctggcttagtcatggatgagactttcaattgctataaagtggttcctttattagacaatgttaccagggaaacaacaggggtttgtttgacttctggggcccacaagtcaacaagagagccccatctaccaaggagcatgtccctgactacccctcagccagcagcaagacatggaccccagtcagggcaggagcagggtttcggcggcgcccagcacaagacattgcccctagagtctcagcccctaccctcgagtaatagatctgcctacctgagactgttgtttgcccaagagctgggtctcagcctgatgggaaccatataaaaaggttcactgacatactgcccacatgttgttctctttcattagatcttagcttccttgtctgctcttcattcttgcagtattcattcaacaaacattaaaaaaaaaaaaaagcattctatgtgtggaacactctgctagatgctgtggatttagaaatgaaaatacatcccgacccttggaatggaagggaaaggactgaagtaagacagattaagcaggaccgtcagcccagcttgaagcccagataaatacggagaacaagagagagcgagtagtgagagatgagtcccaatgcctcactttggtgacgggtgcgtggtgggcttcatgcagcttcttctgataaatgcctccttcagaactggtcaactctaccttggccagtgacccaggtggtcatagtagatttaccaagggaaaatggaaacttttattaggagctcttaggcctcttcacttcatggatttttttttcctttttttttgagatggagttttgccctgtcacccaggctggaatgcagtggtgcaatctcagctcactgcaacctccgcctcccaggttcaagcaattctcctgcctcagcctcccgagtagctgggactacaggtgtgcgccaccacaccaggctaatttttgtattttttgtaaagacaggttttcaccacgttggccaggctggtctgaactccagacctcaggtgattcacctgtctcagcctcccaaagtgctgggattacaggtgtgagccaccgtgcccggctacttcatggatttttgattacagattatgcctcttacaatttttaagaagaatcaagtgggctgaaggtcaatgtcaccataagacaaaagacatttttattagttgattctagggaattggccttaaggggagccctttcttcctaagagattcttaggtgattctcacttcctcttgccccagtattatttttgtttttggtatggctcactcagatccttttttcctcctatccctaagtaatccgggtttctttttcccatatttagaacaaaatgtatttatgcagagtgtgtccaaacctcaacccaaggcctgtatacaaaataaatcaaattaaacacatctttactgtcttctacctctttcctgacctcaatatatcccaacttgcctcactctgagaaccaaggctgtcccagcacctgagtcgcagatattctactgatttgacagaactgtgtgactatctggaacagcattttgatccacaatttgcccagttacaaagcttaaatgagctctagtgcatgcatatatatttcaaaattccaccatgatcttccacactctgtattgtaaatagagccctgtaatgcttttacttcgtatttcattgcttgttatacataaaaatatacttttcttcttcatgttagaaaatgcaaagaataggagggtgggggaatctctgggcttggagacaggagacttgccttcctactatggttccatcagaatgtagactgggacaatacaataattcaagtctggtttgctcatctgtaaattgggaagaatgtttccagctccagaatgctaaatctctaagtctgtggttggcagccactattgcagcagctcttcaatgactcaatgcagttttgcattctccctaccttttttttctaaaaccaataaaatagatacagcctttaggctttctgggatttcccttagtcaagctagggtcatcctgactttcggcgtgaatttgcaaaacaagacctgactctgtactcctgctctaaggactgtgcatggttccaaaggcttagcttgccagcatatttgagctttttccttctgttcaaactgttccaaaatataaaagaataaaattaattaagttggcactggacttccggtggtcagtcatgtgtgtcatctgtcacgtttttcgggctctggtggaaatggatctgtctgtcttctctcataggtggtattcacagccaacgactccggcccccgccgctacaccattgccgccctgctgagcccctactcctattccaccacggctgtcgtcaccaatcccaaggaatgagggacttctcctccagtggacctgaaggacgagggatgggatttcatgtaaccaagagtattccatttttactaaagcagtgttttcacctcatatgctatgttagaagtccaggcagagacaataaaacattcctgtgaaaggcacttttcattccactttaacttgattttttaaattcccttattgtcccttccaaaaaaaagagaatcaaaattttacaaagaatcaaaggaattctagaaagtatctgggcagaacgctaggagagatccaaatttccattgtcttgcaagcaaagcacgtattaaatatgatctgcagccattaaaaagacacattctgtaaatgagagagccttattttcctgtaaccttcagcaaatagcaaaagacacattccaagggcccacttctttactgtgggcactcgagataacttcgtataatgtatgctatacgaagttatatgcatgccagtagcagcacccacgtccaccttctgtctagtaatgtccaacacctccctcagtccaaacactgctctgcatccatgtggctcccatttatacctgaagcacttgatggggcctcaatgttttactagagcccacccccctgcaactctgagaccctctggatttgtctgtcagtgcctcactggggcgttggataatttcttaaaaggtcaagttccctcagcagcattctctgagcagtctgaagatgtgtgcttttcacagttcaaatccatgtggctgtttcacccacctgcctggccttgggttatctatcaggacctagcctagaagcaggtgtgtggcacttaacacctaagctgagtgactaactgaacactcaagtggatgccatctttgtcacttcttgactgtgacacaagcaactcctgatgccaaagccctgcccacccctctcatgcccatatttggacatggtacaggtcctcactggccatggtctgtgaggtcctggtcctctttgacttcataattcctaggggccactagtatctataagaggaagagggtgctggctcccaggccacagcccacaaaattccacctgctcacaggttggctggctcgacccaggtggtgtcccctgctctgagccagctcccggccaagccagcaccatgggaacccccaagaagaagaggaaggtgcgtaccgatttaaattccaatttactgaccgtacaccaaaatttgcctgcattaccggtcgatgcaacgagtgatgaggttcgcaagaacctgatggacatgttcagggatcgccaggcgttttctgagcatacctggaaaatgcttctgtccgtttgccggtcgtgggcggcatggtgcaagttgaataaccggaaatggtttcccgcagaacctgaagatgttcgcgattatcttctatatcttcaggcgcgcggtctggcagtaaaaactatccagcaacatttgggccagctaaacatgcttcatcgtcggtccgggctgccacgaccaagtgacagcaatgctgtttcactggttatgcggcggatccgaaaagaaaacgttgatgccggtgaacgtgcaaaacaggtaaatataaaatttttaagtgtataatgatgttaaactactgattctaattgtttgtgtattttaggctctagcgttcgaacgcactgatttcgaccaggttcgttcactcatggaaaatagcgatcgctgccaggatatacgtaatctggcatttctggggattgcttataacaccctgttacgtatagccgaaattgccaggatcagggttaaagatatctcacgtactgacggtgggagaatgttaatccatattggcagaacgaaaacgctggttagcaccgcaggtgtagagaaggcacttagcctgggggtaactaaactggtcgagcgatggatttccgtctctggtgtagctgatgatccgaataactacctgttttgccgggtcagaaaaaatggtgttgccgcgccatctgccaccagccagctatcaactcgcgccctggaagggatttttgaagcaactcatcgattgatttacggcgctaaggatgactctggtcagagatacctggcctggtctggacacagtgcccgtgtcggagccgcgcgagatatggcccgcgctggagtttcaataccggagatcatgcaagctggtggctggaccaatgtaaatattgtcatgaactatatccgtaacctggatagtgaaacaggggcaatggtgcgcctgctggaagatggcgattaggcggccggccgctaatcagccataccacatttgtagaggttttacttgctttaaaaaacctcccacacctccccctgaacctgaaacataaaatgaatgcaattgttgttgttaacttgtttattgcagcttataatggttacaaataaagcaatagcatcacaaatttcacaaataaagcatttttttcactgcattctagttgtggtttgtccaaactcatcaatgtatcttatcatgtctggatcccccggctagagtttaaacactagaactagtggatcccccgggatcatggcctccgcgccgggttttggcgcctcccgcgggcgcccccctcctcacggcgagcgctgccacgtcagacgaagggcgcagcgagcgtcctgatccttccgcccggacgctcaggacagcggcccgctgctcataagactcggccttagaaccccagtatcagcagaaggacattttaggacgggacttgggtgactctagggcactggttttctttccagagagcggaacaggcgaggaaaagtagtcccttctcggcgattctgcggagggatctccgtggggcggtgaacgccgatgattatataaggacgcgccgggtgtggcacagctagttccgtcgcagccgggatttgggtcgcggttcttgtttgtggatcgctgtgatcgtcacttggtgagtagcgggctgctgggctggccggggctttcgtggccgccgggccgctcggtgggacggaagcgtgtggagagaccgccaagggctgtagtctgggtccgcgagcaaggttgccctgaactgggggttggggggagcgcagcaaaatggcggctgttcccgagtcttgaatggaagacgcttgtgaggcgggctgtgaggtcgttgaaacaaggtggggggcatggtgggcggcaagaacccaaggtcttgaggccttcgctaatgcgggaaagctcttattcgggtgagatgggctggggcaccatctggggaccctgacgtgaagtttgtcactgactggagaactcggtttgtcgtctgttgcgggggcggcagttatggcggtgccgttgggcagtgcacccgtacctttgggagcgcgcgccctcgtcgtgtcgtgacgtcacccgttctgttggcttataatgcagggtggggccacctgccggtaggtgtgcggtaggcttttctccgtcgcaggacgcagggttcgggcctagggtaggctctcctgaatcgacaggcgccggacctctggtgaggggagggataagtgaggcgtcagtttctttggtcggttttatgtacctatcttcttaagtagctgaagctccggttttgaactatgcgctcggggttggcgagtgtgttttgtgaagttttttaggcaccttttgaaatgtaatcatttgggtcaatatgtaattttcagtgttagactagtaaattgtccgctaaattctggccgtttttggcttttttgttagacgtgttgacaattaatcatcggcatagtatatcggcatagtataatacgacaaggtgaggaactaaaccatgggatcggccattgaacaagatggattgcacgcaggttctccggccgcttgggtggagaggctattcggctatgactgggcacaacagacaatcggctgctctgatgccgccgtgttccggctgtcagcgcaggggcgcccggttctttttgtcaagaccgacctgtccggtgccctgaatgaactgcaggacgaggcagcgcggctatcgtggctggccacgacgggcgttccttgcgcagctgtgctcgacgttgtcactgaagcgggaagggactggctgctattgggcgaagtgccggggcaggatctcctgtcatctcaccttgctcctgccgagaaagtatccatcatggctgatgcaatgcggcggctgcatacgcttgatccggctacctgcccattcgaccaccaagcgaaacatcgcatcgagcgagcacgtactcggatggaagccggtcttgtcgatcaggatgatctggacgaagagcatcaggggctcgcgccagccgaactgttcgccaggctcaaggcgcgcatgcccgacggcgatgatctcgtcgtgacccatggcgatgcctgcttgccgaatatcatggtggaaaatggccgcttttctggattcatcgactgtggccggctgggtgtggcggaccgctatcaggacatagcgttggctacccgtgatattgctgaagagcttggcggcgaatgggctgaccgcttcctcgtgctttacggtatcgccgctcccgattcgcagcgcatcgccttctatcgccttcttgacgagttcttctgaggggatccgctgtaagtctgcagaaattgatgatctattaaacaataaagatgtccactaaaatggaagtttttcctgtcatactttgttaagaagggtgagaacagagtacctacattttgaatggaaggattggagctacgggggtgggggtggggtgggattagataaatgcctgctctttactgaaggctctttactattgctttatgataatgtttcatagttggatatcataatttaaacaagcaaaaccaaattaagggccagctcattcctcccactcatgatctatagatctatagatctctcgtgggatcattgtttttctcttgattcccactttgtggttctaagtactgtggtttccaaatgtgtcagtttcatagcctgaagaacgagatcagcagcctctgttccacatacacttcattctcagtattgttttgccaagttctaattccatcagacctcgacctgcagcccctagataacttcgtataatgtatgctatacgaagttatgctaggtaactataacggtcctaaggtagcgagctagcgagactcagcccaggaggaccaggatcttgccaaagcagtagcatcccatttgtaccaaaacagtgttcttgctctataaaccgtgttagcagctcagga

SEQ ID NO: 17 - DNA, 6486 bp, Artificial Sequence
  Synthetic
  misc_feature (1)..(100): Mouse Sequence
  misc_feature (101)..(6308): Human Sequence
  misc_feature (6309)..(6386): Cassette LoxP Scar
  misc_feature (6387)..(6486): Mouse Sequence
atgtacttttggttttgttccagagtctatcaccggaaagaacaagccggtttactctgacccatttcactgacatttctcttgtctcctctgtgcccagggcaccggtgaatccaagtgtcctctgatggtcaaagttctagatgctgtccgaggcagtcctgccatcaatgtggccgtgcatgtgttcagaaaggctgctgatgacacctgggagccatttgcctctgggtaagttgccaaagaaccctcccacaggacttggttttatcttcccgtttgcccctcacttggtagagagaggctcacatcatctgctaaagaatttacaagtagattgaaaaacgtaggcagaggtcaagtatgccctctgaaggatgccctctttttgttttgcttagctaggaagtgaccaggaacctgagcatcatttaggggcagacagtagagaaaagaaggaatcagaactcctctcctctagctgtggtttgcaacccttttgggtcacagaacactttatgtaggtgatgaaaagtaaacattctatgcccagaaaaaatgcacagatacacacacatacaaaatcatatatgtgattttaggagtttcacagattccctggtgtccctgggtaacaccaaagctaagtgtccttgtcttagaattttaggaaaaggtataatgtgtattaacccattaacaaaaggaaaggaattcagaaatattattaaccaggcatctgtctgtagttaatatggatcacccaaaacccaaggcttttgcctaatgaacactttggggcacctactgtgtgcaaggctgggggctgtcaagctcagttaaaaaaaaaaagatagaagagatggatccatgaggcaaagtacagccccaggctaatcccacgatcacccgacttcatgtccaagagtggcttctcaccttcattagccagttcacaattttcatggagtttttctacctgcactagcaaaaacttcaaggaaaatacatattaataaatctaagcaaagtgaccagaagacagagcaatcaggagaccctttgcatccagcagaagaggaactgctaagtatttacatctccacagagaagaatttctgttgggttttaattgaaccccaagaaccacatgattcttcaaccattattgggaagatcattttcttaggtctggttttaactggctttttatttgggaattcatttatgtttatataaaatgccaagcataacatgaaaagtggttacaggactattctaagggagagacagaatggacaccaaaaatattccaatgttcttgtgaatcttttccttgcaccaggacaaaaaaaaaaagaagtgaaaagaagaaaggaggaggggcataatcagagtcagtaaagacaactgctatttttatctatcgtagctgttgcagtcaaatgggaagcaatttccaacattcaactatggagctggtacttacatggaaatagaagttgcctagtgtttgttgctggcaaagagttatcagagaggttaaatatataaaagggaaaagagtcagatacaggttcttcttcctactttaggttttccactgtgtgtgcaaatgatactccctggtggtgtgcagatgcctcaaagctatcctcacaccacaagggagaggagcgagatcctgctgtcctggagaagtgcagagttagaacagctgtggccacttgcatccaatcatcaatcttgaatcacagggactctttcttaagtaaacattatacctggccgggcacggtggctcacgcctgtaatcccagcactttgggatgccaaagtgggcatatcatctgaggtcaggagttcaagaccagcctggccaacatggcaaaactccgtctttatgaaaaatacaaaaattagccaggcatggtggcaggcgcctgtaatcccagctaattgggaggctgaggctggagaatcccttgaatctaggaggcagaggttgcagtgagctgagatcgtgccattgcactccagcctgggtgacaagagtaaaactctgtctcaaaaaaaaaaaattatacctacattctcttcttatcagagaaaaaaatctacagtgagcttttcaaaaagtttttacaaactttttgccatttaatttcagttaggagttttccctacttctgacttagttgaggggaaatgttcataacatgtttataacatgtttatgtgtgttagttggtgggggtgtattactttgccatgccatttgtttcctccatgcgtaacttaatccagactttcacaccttataggaaaaccagtgagtctggagagctgcatgggctcacaactgaggaggaatttgtagaagggatatacaaagtggaaatagacaccaaatcttactggaaggcacttggcatctccccattccatgagcatgcagaggtgagtatacagaccttcgagggttgttttggttttggtttttgcttttggcattccaggaaatgcacagttttactcagtgtaccacagaaatgtcctaaggaaggtgatgaatgaccaaaggttccctttcctattatacaagaaaaaattcacaacactctgagaagcaaatttctttttgactttgatgaaaatccacttagtaacatgacttgaacttacatgaaactactcatagtctattcattccactttatatgaatattgatgtatctgctgttgaaataatagtttatgaggcagccctccagaccccacgtagagtgtatgtaacaagagatgcaccattttatttctcgaaaacccgtaacattcttcattccaaaacacatctggcttctcggaggtctggacaagtgattcttggcaacacatacctatagagacaataaaatcaaagtaataatggcaacacaatagataacatttaccaagcatacaccatgtggcagacacaattataagtgttttccatatttaacctacttaatcctcaggaataagccactgaggtcagtcctattattatccccatcttatagatgaagaaaatgaggcaccaggaagtcaaataacttgtcaaaggtcacaagactaggaaatacacaagtagaaatgtttacaattaaggcccaggctgggtttgccctcagttctgctatgcctcgcattatgccccaggaaactttttcccttgtgaaagccaagcttaaaaaaagaaaagccacatttgtaacgtgctctgttcccctgcctatggtgaggatcttcaaacagttatacatggacccagtccccctgccttctccttaatttcttaagtcatttgaaacagatggctgtcatggaaatagaatccagacatgttggtcagagttaaagatcaactaattccatcaaaaatagctcggcatgaaagggaactattctctggcttagtcatggatgagactttcaattgctataaagtggttcctttattagacaatgttaccagggaaacaacaggggtttgtttgacttctggggcccacaagtcaacaagagagccccatctaccaaggagcatgtccctgactacccctcagccagcagcaagacatggaccccagtcagggcaggagcagggtttcggcggcgcccagcacaagacattgcccctagagtctcagcccctaccctcgagtaatagatctgcctacctgagactgttgtttgcccaagagctgggtctcagcctgatgggaaccatataaaaaggttcactgacatactgcccacatgttgttctctttcattagatcttagcttccttgtctgctcttcattcttgcagtattcattcaacaaacattaaaaaaaaaaaaaagcattctatgtgtggaacactctgctagatgctgtggatttagaaatgaaaatacatcccgacccttggaatggaagggaaaggactgaagtaagacagattaagcaggaccgtcagcccagcttgaagcccagataaatacggagaacaagagagagcgagtagtgagagatgagtcccaatgcctcactttggtgacgggtgcgtggtgggcttcatgcagcttcttctgataaatgcctccttcagaactggtcaactctaccttggccagtgacccaggtggtcatagtagatttaccaagggaaaatggaaacttttattaggagctcttaggcctcttcacttcatggatttttttttcctttttttttgagatggagttttgccctgtcacccaggctggaatgcagtggtgcaatctcagctcactgcaacctccgcctcccaggttcaagcaattctcctgcctcagcctcccgagtagctgggactacaggtgtgcgccaccacaccaggctaatttttgtattttttgtaaagacaggttttcaccacgttggccaggctggtctgaactccagacctcaggtgattcacctgtctcagcctcccaaagtgctgggattacaggtgtgagccaccgtgcccggctacttcatggatttttgattacagattatgcctcttacaatttttaagaagaatcaagtgggctgaaggtcaatgtcaccataagacaaaagacatttttattagttgattctagggaattggccttaaggggagccctttcttcctaagagattcttaggtgattctcacttcctcttgccccagtattatttttgtttttggtatggctcactcagatccttttttcctcctatccctaagtaatccgggtttctttttcccatatttagaacaaaatgtatttatgcagagtgtgtccaaacctcaacccaaggcctgtatacaaaataaatcaaattaaacacatctttactgtcttctacctctttcctgacctcaatatatcccaacttgcctcactctgagaaccaaggctgtcccagcacctgagtcgcagatattctactgatttgacagaactgtgtgactatctggaacagcattttgatccacaatttgcccagttacaaagcttaaatgagctctagtgcatgcatatatatttcaaaattccaccatgatcttccacactctgtattgtaaatagagccctgtaatgcttttacttcgtatttcattgcttgttatacataaaaatatacttttcttcttcatgttagaaaatgcaaagaataggagggtgggggaatctctgggcttggagacaggagacttgccttcctactatggttccatcagaatgtagactgggacaatacaataattcaagtctggtttgctcatctgtaaattgggaagaatgtttccagctccagaatgctaaatctctaagtctgtggttggcagccactattgcagcagctcttcaatgactcaatgcagttttgcattctccctaccttttttttctaaaaccaataaaatagatacagcctttaggctttctgggatttcccttagtcaagctagggtcatcctgactttcggcgtgaatttgcaaaacaagacctgactctgtactcctgctctaaggactgtgcatggttccaaaggcttagcttgccagcatatttgagctttttccttctgttcaaactgttccaaaatataaaagaataaaattaattaagttggcactggacttccggtggtcagtcatgtgtgtcatctgtcacgtttttcgggctctggtggaaatggatctgtctgtcttctctcataggtggtattcacagccaacgactccggcccccgccgctacaccattgccgccctgctgagcccctactcctattccaccacggctgtcgtcaccaatcccaaggaatgagggacttctcctccagtggacctgaaggacgagggatgggatttcatgtaaccaagagtattccatttttactaaagcagtgttttcacctcatatgctatgttagaagtccaggcagagacaataaaacattcctgtgaaaggcacttttcattccactttaacttgattttttaaattcccttattgtcccttccaaaaaaaagagaatcaaaattttacaaagaatcaaaggaattctagaaagtatctgggcagaacgctaggagagatccaaatttccattgtcttgcaagcaaagcacgtattaaatatgatctgcagccattaaaaagacacattctgtaaatgagagagccttattttcctgtaaccttcagcaaatagcaaaagacacattccaagggcccacttctttactgtgggcactcgagataacttcgtataatgtatgctatacgaagttatgctaggtaactataacggtcctaaggtagcgagctagcgagactcagcccaggaggaccaggatcttgccaaagcagtagcatcccatttgtaccaaaacagtgttcttgctctataaaccgtgttagcagctcagga

SEQ ID NO: 18 - DNA, 7201 bp, Homo sapiens
atggcttctcatcgtctgctcctcctctgccttgctggactggtatttgtgtctgaggctggccctacggtgagtgtttctgtgacatcccattcctacatttaagattcacgctaaatgaagtagaagtgactccttccagctttgccaaccagcttttattactagggcaagggtacccagcatctatttttaatataattaattcaaacttcaaaaagaatgaagttccactgagcttactgagctgggacttgaactctgagcattctacctcattgctttggtgcattaggtttgtaatatctggtacctctgtttcctcagatagatgatagaaataaagatatgatattaaggaagctgttaatactgaattttcagaaaagtatccctccataaaatgtatttgggggacaaactgcaggagattatattctggccctatagttattcaaaacgtatttattgattaatctttaaaaggcttagtgaacaatattctagtcagatatctaattcttaaatcctctagaagaattaactaatactataaaatgggtctggatgtagttctgacattattttataacaactggtaagagggagtgactatagcaacaactaaaatgatctcaggaaaacctgtttggccctatgtatggtacattacatcttttcagtaattccactcaaatggagacttttaacaaagcaactgttctcaggggacctattttctcccttaaaattcattatacacatccctggttgatagcagtgtgtctggaggcagaaaccattcttgctttggaaacaattacgtctgtgttatactgagtagggaagctcattaattgtcgacacttacgttcctgataatgggatcagtgtgtaattcttgtttcgctccagatttctaataccacaaagaataaatcctttcactctgatcaattttgttaacttctcacgtgtcttctctacacccagggcaccggtgaatccaagtgtcctctgatggtcaaagttctagatgctgtccgaggcagtcctgccatcaatgtggccgtgcatgtgttcagaaaggctgctgatgacacctgggagccatttgcctctgggtaagttgccaaagaaccctcccacaggacttggttttatcttcccgtttgcccctcacttggtagagagaggctcacatcatctgctaaagaatttacaagtagattgaaaaacgtaggcagaggtcaagtatgccctctgaaggatgccctctttttgttttgcttagctaggaagtgaccaggaacctgagcatcatttaggggcagacagtagagaaaagaaggaatcagaactcctctcctctagctgtggtttgcaacccttttgggtcacagaacactttatgtaggtgatgaaaagtaaacattctatgcccagaaaaaatgcacagatacacacacatacaaaatcatatatgtgattttaggagtttcacagattccctggtgtccctgggtaacaccaaagctaagtgtccttgtcttagaattttaggaaaaggtataatgtgtattaacccattaacaaaaggaaaggaattcagaaatattattaaccaggcatctgtctgtagttaatatggatcacccaaaacccaaggcttttgcctaatgaacactttggggcacctactgtgtgcaaggctgggggctgtcaagctcagttaaaaaaaaaaagatagaagagatggatccatgaggcaaagtacagccccaggctaatcccacgatcacccgacttcatgtccaagagtggcttctcaccttcattagccagttcacaattttcatggagtttttctacctgcactagcaaaaacttcaaggaaaatacatattaataaatctaagcaaagtgaccagaagacagagcaatcaggagaccctttgcatccagcagaagaggaactgctaagtatttacatctccacagagaagaatttctgttgggttttaattgaaccccaagaaccacatgattcttcaaccattattgggaagatcattttcttaggtctggttttaactggctttttatttgggaattcatttatgtttatataaaatgccaagcataacatgaaaagtggttacaggactattctaagggagagacagaatggacaccaaaaatattccaatgttcttgtgaatcttttccttgcaccaggacaaaaaaaaaaagaagtgaaaagaagaaaggaggaggggcataatcagagtcagtaaagacaactgctatttttatctatcgtagctgttgcagtcaaatgggaagcaatttccaacattcaactatggagctggtacttacatggaaatagaagttgcctagtgtttgttgctggcaaagagttatcagagaggttaaatatataaaagggaaaagagtcagatacaggttcttcttcctactttaggttttccactgtgtgtgcaaatgatactccctggtggtgtgcagatgcctcaaagctatcctcacaccacaagggagaggagcgagatcctgctgtcctggagaagtgcagagttagaacagctgtggccacttgcatccaatcatcaatcttgaatcacagggactctttcttaagtaaacattatacctggccgggcacggtggctcacgcctgtaatcccagcactttgggatgccaaagtgggcatatcatctgaggtcaggagttcaagaccagcctggccaacatggcaaaactccgtctttatgaaaaatacaaaaattagccaggcatggtggcaggcgcctgtaatcccagctaattgggaggctgaggctggagaatcccttgaatctaggaggcagaggttgcagtgagctgagatcgtgccattgcactccagcctgggtgacaagagtaaaactctgtctcaaaaaaaaaaaattatacctacattctcttcttatcagagaaaaaaatctacagtgagcttttcaaaaagtttttacaaactttttgccatttaatttcagttaggagttttccctacttctgacttagttgaggggaaatgttcataacatgtttataacatgtttatgtgtgttagttggtgggggtgtattactttgccatgccatttgtttcctccatgcgtaacttaatccagactttcacaccttataggaaaaccagtgagtctggagagctgcatgggctcacaactgaggaggaatttgtagaagggatatacaaagtggaaatagacaccaaatcttactggaaggcacttggcatctccccattccatgagcatgcagaggtgagtatacagaccttcgagggttgttttggttttggtttttgcttttggcattccaggaaatgcacagttttactcagtgtaccacagaaatgtcctaaggaaggtgatgaatgaccaaaggttccctttcctattatacaagaaaaaattcacaacactctgagaagcaaatttctttttgactttgatgaaaatccacttagtaacatgacttgaacttacatgaaactactcatagtctattcattccactttatatgaatattgatgtatctgctgttgaaataatagtttatgaggcagccctccagaccccacgtagagtgtatgtaacaagagatgcaccattttatttctcgaaaacccgtaacattcttcattccaaaacacatctggcttctcggaggtctggacaagtgattcttggcaacacatacctatagagacaataaaatcaaagtaataatggcaacacaatagataacatttaccaagcatacaccatgtggcagacacaattataagtgttttccatatttaacctacttaatcctcaggaataagccactgaggtcagtcctattattatccccatcttatagatgaagaaaatgaggcaccaggaagtcaaataacttgtcaaaggtcacaagactaggaaatacacaagtagaaatgtttacaattaaggcccaggctgggtttgccctcagttctgctatgcctcgcattatgccccaggaaactttttcccttgtgaaagccaagcttaaaaaaagaaaagccacatttgtaacgtgctctgttcccctgcctatggtgaggatcttcaaacagttatacatggacccagtccccctgccttctccttaatttcttaagtcatttgaaacagatggctgtcatggaaatagaatccagacatgttggtcagagttaaagatcaactaattccatcaaaaatagctcggcatgaaagggaactattctctggcttagtcatggatgagactttcaattgctataaagtggttcctttattagacaatgttaccagggaaacaacaggggtttgtttgacttctggggcccacaagtcaacaagagagccccatctaccaaggagcatgtccctgactacccctcagccagcagcaagacatggaccccagtcagggcaggagcagggtttcggcggcgcccagcacaagacattgcccctagagtctcagcccctaccctcgagtaatagatctgcctacctgagactgttgtttgcccaagagctgggtctcagcctgatgggaaccatataaaaaggttcactgacatactgcccacatgttgttctctttcattagatcttagcttccttgtctgctcttcattcttgcagtattcattcaacaaacattaaaaaaaaaaaaaagcattctatgtgtggaacactctgctagatgctgtggatttagaaatgaaaatacatcccgacccttggaatggaagggaaaggactgaagtaagacagattaagcaggaccgtcagcccagcttgaagcccagataaatacggagaacaagagagagcgagtagtgagagatgagtcccaatgcctcactttggtgacgggtgcgtggtgggcttcatgcagcttcttctgataaatgcctccttcagaactggtcaactctaccttggccagtgacccaggtggtcatagtagatttaccaagggaaaatggaaacttttattaggagctcttaggcctcttcacttcatggatttttttttcctttttttttgagatggagttttgccctgtcacccaggctggaatgcagtggtgcaatctcagctcactgcaacctccgcctcccaggttcaagcaattctcctgcctcagcctcccgagtagctgggactacaggtgtgcgccaccacaccaggctaatttttgtattttttgtaaagacaggttttcaccacgttggccaggctggtctgaactccagacctcaggtgattcacctgtctcagcctcccaaagtgctgggattacaggtgtgagccaccgtgcccggctacttcatggatttttgattacagattatgcctcttacaatttttaagaagaatcaagtgggctgaaggtcaatgtcaccataagacaaaagacatttttattagttgattctagggaattggccttaaggggagccctttcttcctaagagattcttaggtgattctcacttcctcttgccccagtattatttttgtttttggtatggctcactcagatccttttttcctcctatccctaagtaatccgggtttctttttcccatatttagaacaaaatgtatttatgcagagtgtgtccaaacctcaacccaaggcctgtatacaaaataaatcaaattaaacacatctttactgtcttctacctctttcctgacctcaatatatcccaacttgcctcactctgagaaccaaggctgtcccagcacctgagtcgcagatattctactgatttgacagaactgtgtgactatctggaacagcattttgatccacaatttgcccagttacaaagcttaaatgagctctagtgcatgcatatatatttcaaaattccaccatgatcttccacactctgtattgtaaatagagccctgtaatgcttttacttcgtatttcattgcttgttatacataaaaatatacttttcttcttcatgttagaaaatgcaaagaataggagggtgggggaatctctgggcttggagacaggagacttgccttcctactatggttccatcagaatgtagactgggacaatacaataattcaagtctggtttgctcatctgtaaattgggaagaatgtttccagctccagaatgctaaatctctaagtctgtggttggcagccactattgcagcagctcttcaatgactcaatgcagttttgcattctccctaccttttttttctaaaaccaataaaatagatacagcctttaggctttctgggatttcccttagtcaagctagggtcatcctgactttcggcgtgaatttgcaaaacaagacctgactctgtactcctgctctaaggactgtgcatggttccaaaggcttagcttgccagcatatttgagctttttccttctgttcaaactgttccaaaatataaaagaataaaattaattaagttggcactggacttccggtggtcagtcatgtgtgtcatctgtcacgtttttcgggctctggtggaaatggatctgtctgtcttctctcataggtggtattcacagccaacgactccggcccccgccgctacaccattgccgccctgctgagcccctactcctattccaccacggctgtcgtcaccaatcccaaggaatgagggacttctcctccagtggacctgaaggacgagggatgggatttcatgtaaccaagagtattccatttttactaaagcagtgttttcacctcatatgctatgttagaagtccaggcagagacaataaaacattcctgtgaaaggcacttttcattccactttaacttgattttttaaattcccttattgtcccttccaaaaaaaagagaatcaaaattttacaaagaatcaaaggaattctagaaagtatctgggcagaacgctaggagagatccaaatttccattgtcttgcaagcaaagcacgtattaaatatgatctgcagccattaaaaagacacattctgtaaatgagagagccttattttcctgtaaccttcagcaaatagcaaaagacacattccaagggcccacttctttactgtgggca

SEQ ID NO: 19 - DNA, 6208 bp, Homo sapiens
ggcaccggtgaatccaagtgtcctctgatggtcaaagttctagatgctgtccgaggcagtcctgccatcaatgtggccgtgcatgtgttcagaaaggctgctgatgacacctgggagccatttgcctctgggtaagttgccaaagaaccctcccacaggacttggttttatcttcccgtttgcccctcacttggtagagagaggctcacatcatctgctaaagaatttacaagtagattgaaaaacgtaggcagaggtcaagtatgccctctgaaggatgccctctttttgttttgcttagctaggaagtgaccaggaacctgagcatcatttaggggcagacagtagagaaaagaaggaatcagaactcctctcctctagctgtggtttgcaacccttttgggtcacagaacactttatgtaggtgatgaaaagtaaacattctatgcccagaaaaaatgcacagatacacacacatacaaaatcatatatgtgattttaggagtttcacagattccctggtgtccctgggtaacaccaaagctaagtgtccttgtcttagaattttaggaaaaggtataatgtgtattaacccattaacaaaaggaaaggaattcagaaatattattaaccaggcatctgtctgtagttaatatggatcacccaaaacccaaggcttttgcctaatgaacactttggggcacctactgtgtgcaaggctgggggctgtcaagctcagttaaaaaaaaaaagatagaagagatggatccatgaggcaaagtacagccccaggctaatcccacgatcacccgacttcatgtccaagagtggcttctcaccttcattagccagttcacaattttcatggagtttttctacctgcactagcaaaaacttcaaggaaaatacatattaataaatctaagcaaagtgaccagaagacagagcaatcaggagaccctttgcatccagcagaagaggaactgctaagtatttacatctccacagagaagaatttctgttgggttttaattgaaccccaagaaccacatgattcttcaaccattattgggaagatcattttcttaggtctggttttaactggctttttatttgggaattcatttatgtttatataaaatgccaagcataacatgaaaagtggttacaggactattctaagggagagacagaatggacaccaaaaatattccaatgttcttgtgaatcttttccttgcaccaggacaaaaaaaaaaagaagtgaaaagaagaaaggaggaggggcataatcagagtcagtaaagacaactgctatttttatctatcgtagctgttgcagtcaaatgggaagcaatttccaacattcaactatggagctggtacttacatggaaatagaagttgcctagtgtttgttgctggcaaagagttatcagagaggttaaatatataaaagggaaaagagtcagatacaggttcttcttcctactttaggttttccactgtgtgtgcaaatgatactccctggtggtgtgcagatgcctcaaagctatcctcacaccacaagggagaggagcgagatcctgctgtcctggagaagtgcagagttagaacagctgtggccacttgcatccaatcatcaatcttgaatcacagggactctttcttaagtaaacattatacctggccgggcacggtggctcacgcctgtaatcccagcactttgggatgccaaagtgggcatatcatctgaggtcaggagttcaagaccagcctggccaacatggcaaaactccgtctttatgaaaaatacaaaaattagccaggcatggtggcaggcgcctgtaatcccagctaattgggaggctgaggctggagaatcccttgaatctaggaggcagaggttgcagtgagctgagatcgtgccattgcactccagcctgggtgacaagagtaaaactctgtctcaaaaaaaaaaaattatacctacattctcttcttatcagagaaaaaaatctacagtgagcttttcaaaaagtttttacaaactttttgccatttaatttcagttaggagttttccctacttctgacttagttgaggggaaatgttcataacatgtttataacatgtttatgtgtgttagttggtgggggtgtattactttgccatgccatttgtttcctccatgcgtaacttaatccagactttcacaccttataggaaaaccagtgagtctggagagctgcatgggctcacaactgaggaggaatttgtagaagggatatacaaagtggaaatagacaccaaatcttactggaaggcacttggcatctccccattccatgagcatgcagaggtgagtatacagaccttcgagggttgttttggttttggtttttgcttttggcattccaggaaatgcacagttttactcagtgtaccacagaaatgtcctaaggaaggtgatgaatgaccaaaggttccctttcctattatacaagaaaaaattcacaacactctgagaagcaaatttctttttgactttgatgaaaatccacttagtaacatgacttgaacttacatgaaactactcatagtctattcattccactttatatgaatattgatgtatctgctgttgaaataatagtttatgaggcagccctccagaccccacgtagagtgtatgtaacaagagatgcaccattttatttctcgaaaacccgtaacattcttcattccaaaacacatctggcttctcggaggtctggacaagtgattcttggcaacacatacctatagagacaataaaatcaaagtaataatggcaacacaatagataacatttaccaagcatacaccatgtggcagacacaattataagtgttttccatatttaacctacttaatcctcaggaataagccactgaggtcagtcctattattatccccatcttatagatgaagaaaatgaggcaccaggaagtcaaataacttgtcaaaggtcacaagactaggaaatacacaagtagaaatgtttacaattaaggcccaggctgggtttgccctcagttctgctatgcctcgcattatgccccaggaaactttttcccttgtgaaagccaagcttaaaaaaagaaaagccacatttgtaacgtgctctgttcccctgcctatggtgaggatcttcaaacagttatacatggacccagtccccctgccttctccttaatttcttaagtcatttgaaacagatggctgtcatggaaatagaatccagacatgttggtcagagttaaagatcaactaattccatcaaaaatagctcggcatgaaagggaactattctctggcttagtcatggatgagactttcaattgctataaagtggttcctttattagacaatgttaccagggaaacaacaggggtttgtttgacttctggggcccacaagtcaacaagagagccccatctaccaaggagcatgtccctgactacccctcagccagcagcaagacatggaccccagtcagggcaggagcagggtttcggcggcgcccagcacaagacattgcccctagagtctcagcccctaccctcgagtaatagatctgcctacctgagactgttgtttgcccaagagctgggtctcagcctgatgggaaccatataaaaaggttcactgacatactgcccacatgttgttctctttcattagatcttagcttccttgtctgctcttcattcttgcagtattcattcaacaaacattaaaaaaaaaaaaaagcattctatgtgtggaacactctgctagatgctgtggatttagaaatgaaaatacatcccgacccttggaatggaagggaaaggactgaagtaagacagattaagcaggaccgtcagcccagcttgaagcccagataaatacggagaacaagagagagcgagtagtgagagatgagtcccaatgcctcactttggtgacgggtgcgtggtgggcttcatgcagcttcttctgataaatgcctccttcagaactggtcaactctaccttggccagtgacccaggtggtcatagtagatttaccaagggaaaatggaaacttttattaggagctcttaggcctcttcacttcatggatttttttttcctttttttttgagatggagttttgccctgtcacccaggctggaatgcagtggtgcaatctcagctcactgcaacctccgcctcccaggttcaagcaattctcctgcctcagcctcccgagtagctgggactacaggtgtgcgccaccacaccaggctaatttttgtattttttgtaaagacaggttttcaccacgttggccaggctggtctgaactccagacctcaggtgattcacctgtctcagcctcccaaagtgctgggattacaggtgtgagccaccgtgcccggctacttcatggatttttgattacagattatgcctcttacaatttttaagaagaatcaagtgggctgaaggtcaatgtcaccataagacaaaagacatttttattagttgattctagggaattggccttaaggggagccctttcttcctaagagattcttaggtgattctcacttcctcttgccccagtattatttttgtttttggtatggctcactcagatccttttttcctcctatccctaagtaatccgggtttctttttcccatatttagaacaaaatgtatttatgcagagtgtgtccaaacctcaacccaaggcctgtatacaaaataaatcaaattaaacacatctttactgtcttctacctctttcctgacctcaatatatcccaacttgcctcactctgagaaccaaggctgtcccagcacctgagtcgcagatattctactgatttgacagaactgtgtgactatctggaacagcattttgatccacaatttgcccagttacaaagcttaaatgagctctagtgcatgcatatatatttcaaaattccaccatgatcttccacactctgtattgtaaatagagccctgtaatgcttttacttcgtatttcattgcttgttatacataaaaatatacttttcttcttcatgttagaaaatgcaaagaataggagggtgggggaatctctgggcttggagacaggagacttgccttcctactatggttccatcagaatgtagactgggacaatacaataattcaagtctggtttgctcatctgtaaattgggaagaatgtttccagctccagaatgctaaatctctaagtctgtggttggcagccactattgcagcagctcttcaatgactcaatgcagttttgcattctccctaccttttttttctaaaaccaataaaatagatacagcctttaggctttctgggatttcccttagtcaagctagggtcatcctgactttcggcgtgaatttgcaaaacaagacctgactctgtactcctgctctaaggactgtgcatggttccaaaggcttagcttgccagcatatttgagctttttccttctgttcaaactgttccaaaatataaaagaataaaattaattaagttggcactggacttccggtggtcagtcatgtgtgtcatctgtcacgtttttcgggctctggtggaaatggatctgtctgtcttctctcataggtggtattcacagccaacgactccggcccccgccgctacaccattgccgccctgctgagcccctactcctattccaccacggctgtcgtcaccaatcccaaggaatgagggacttctcctccagtggacctgaaggacgagggatgggatttcatgtaaccaagagtattccatttttactaaagcagtgttttcacctcatatgctatgttagaagtccaggcagagacaataaaacattcctgtgaaaggcacttttcattccactttaacttgattttttaaattcccttattgtcccttccaaaaaaaagagaatcaaaattttacaaagaatcaaaggaattctagaaagtatctgggcagaacgctaggagagatccaaatttccattgtcttgcaagcaaagcacgtattaaatatgatctgcagccattaaaaagacacattctgtaaatgagagagccttattttcctgtaaccttcagcaaatagcaaaagacacattccaagggcccacttctttactgtgggca

SEQ ID NO: 20 - DNA, 8300 bp, Mus musculus
atggcttcccttcgactcttcctcctttgcctcgctggactggtatttgtgtctgaagctggccccgcggtgagtgatcctgtgagcgatccagacatggcagttagaccttagataaagaagaagtgccttcttccagatgtgagaactagagtactcagactctatatttaccattagactccaaagagaagagctggagtgcctctggctcttccttctattgctttagcgcattgggtctgtagtgctcagtctctggtgtccttagataataaagatatgagattaacatagaaataaagatataaaagggctggatgtatagtttagtggtccagtgtatgcctagtatgtgaaaagccttctgttcaacctctagcaatagaaaaacaagatatattctcggtggggctgttaatattgaattctcataaaatctttaatatatttagtatgcctattatgttgttatattttagttctttagctaatcaaaatgcattattgatctttctttgtctttttttggccaacactctattccagtctttgaaaaagtcctttaaaagagttaatcagtataattaaatgagtcaggaagtatgtgagggttattttacaaccagagggaattactatagcaacagctgattagaatgatctcaagaaaaagcccattctgtctttttgcaccatgcacctttcagtggctccattcagatggagaggcaaacagagcaatggctctcagagggcctattttccctttgaacattcattatccatatccctggtgcacagcagtgcatctgggggcagaaactgttcttgctttggaaacaatgctgtctatgtcatactggataaagaagctcattaattgtcaacacttatgttatcataatgggatcagcatgtacttttggttttgttccagagtctatcaccggaaagaacaagccggtttactctgacccatttcactgacatttctcttgtctcctctgtgcccagggtgctggagaatccaaatgtcctctgatggtcaaagtcctggatgctgtccgaggcagccctgctgtagacgtggctgtaaaagtgttcaaaaagacctctgagggatcctgggagccctttgcctctgggtaagcttgtagaaagcccaccatgggaccggttccaggttcccatttgctcttattcgtgttagattcagacacacacaacttaccagctagagggctcagagagagggctcaggggcgaagggcacgtattgctcttgtaagagacacaggtttaattcctagcaccagaatggcagctcataaccatctgaaactcacagtcttaggagatctgggtatctgacattctcttctacccaccatgtgtgtggtgcacaaattcacatgcaggcatcaaatcttataaacaacaacaaaaaaccaacaaacctggtagcaaaagaagattagaaggttaaacatatgagccgagagcttttgttttgttttgttttgttttgttttgtttacatttcaaatgttatcccctttctcggtccccctccccaaaccctctaccccattctctcctccccttcttctatgagggtgttccccaccaacccactcccaccttcctgctctcgaattcccctatactgggacatcaagccttcacagaatcaagggcctctcctcccattgatgcccgacaatgtcatcctctgctacctatgtggctggagccatgggtcccttcatgtatcctccttggttggtggtttagtctctgggaggtctgggggatctggttgattgatattattgttcttcctatgagattgcaaaccccttcagctccttcggtcctttaactcctccactggggaccccgagctcagtccaatggttggctgtgagcatccaccagcagaggcctttttttttttttttaacaaagctgctttattatgttgcttagagcatgaccaggaaccagagcacagtccaagactgaagggaggaaaagggggggagtcaataaccccactgtttcatagtggtttgcaacccttttatatcacagcccactttaggcaaataatgaaaattatagtctccagggacagagaagatggtgcaggaagtgaagtgcctgctcagaaaatgggggcttgaatgtgagttcccagactctgtgtaagatgcccagcatcgaagtgcatgcttataacaccagcctggaggtagaagcttagaaacaggggtaccctgaagttgcttgttcaccagtgtccctgaatgggtaggtgcatgtttggtgagagaccctgtctcaaaaatcaaggtgtaggataattgaaaatacctagctttgagcttagatcatgcaaatgtgtacacacactcacacacaccacacacacaaaaaaatgcagagacagagagatacagagagacagagagatacagagacagagacagagagaaaaggagaaagtaaaaaacaaataatttaaagacccatggccacaaagaggctcaaagacaagcacgtataaaaccatacacatgtaattttaggagttttcagattccctggtacccgtgggtgatgcacaagctttgaatcccagtcttaaaatcttacgaagaacgtgttcgtgtgtgctaatttattgatgagaggaaaggaattgacaaagtgcccttccggagcttcctgcattacccagactcagggtttttttaaatgtacactcagaacagagtagctctgtgcaagggtagcaaccacgaagcttaataagaaacatatcgtgagagatctgcaaggcaaatctaggggctgaccaatctcacagtcacccactagcatgtcaacacaacttcccacctgtgctagccacttagcaattttgtgttgttctgttttgtttttgtttttaacaaagcaatttcaaagagatttctaattcatctaaacaaacaaaccaaaaggaaaacagcaaagacgccctgagcacttagcagagcagctatgcagttatgactcctgggtggagactttatatcaggcttcaactgaatacctagaacctactagtgctcttcatcaatccttgggaaggtcattttcttttggtgctgttttgagtttctatttgttaatgtcttcataattatacacgtgttgagcacagcatgcaaagtgattaggggaatctagttggagtggaatggatacccaaatattcagactttcttgtgactcttctttcttgtacccacatcaaaaaaaaaaaaaatggagatgagacatggtcagagtcactaaaaccagctgctacttttaattacgtggggagcagtttctaacattgccattattgaactgatgctgcctgggtggaaatggaaatcacttagtatttcttgttggcaaagaattactgaatggattaaatttccaaagggagaagtcagttacaagtcttttctttgtttattaggctttctgctatgataaattacactacttccagaagttacccttaggccatgggacactggactatcactctgctgtcacaagagattacagagttagtcaaggcagcttgtgacaccttcagggactgtcataaacttccagcaagtcattaatcctgaatgcaatactgtgtgtgtgtgtctatgtgtgtttgtatgtctgtgtgtgtcttatgtctgtgtctctgtgtgtgtgtgtgtttgtgtgtgtgtgtgtatgtatgcctgtgtgtgtcttatgtctgtgtttgtgtgtctgtgtgtgtcttatgtctgtgtttgtatgtctgtgtgtgtctgtgtgtgtcttatgtctgtgtctctgtgtgtgtgtgtgtgtatgtatgtatgtatgtatgtatgtgtatgtgtttgcatctctctgtgtgtctgcgcttatatatttgtgtatgtgtttatgtgttcgcctttgtgcgttgttggggattgaatccaggggaatacaaatgttaagaaagaacgttaccactaagcttcacctgtaggccttaaagcttttctttcttttaaaaattgtaattaattcattttcagtcaggatctccacacctcgtccctgctgctctagaactcactatttaaacacaatcgccctcaaacctgcagcaaccctcccgcctctaccctgcgagcactagaataataacaggtgaccccacacgcctagattaagacctttaaggtaaacattttactatattttagtctcataagacaagatgctacaataaagctgtacataaagttccctcgaatttcttgctattttaactcaaacataaggatttcctcctttttgattcaggtaacagaaaaaatacacaggtacatacatgtacacacatgaacacacacgcatcacaaccacatatgcgcacgcttgtgtgatctatcatttaccatgccactgaactcttctttccccataaattcctctggacttgtgtgccctccaggaagaccgcggagtctggagagctgcacgggctcaccacagatgagaagtttgtagaaggagtgtacagagtagaactggacaccaaatcgtactggaagacacttggcatttccccgttccatgaattcgcggatgtaagtggacacaccaagttgtttggattttgtttttagtctcaggaaattcccttcgctcttgctgtacgatgggcatgagtggaaagtagattccacagccagaatccacagtgctgggaaagcaagccttctgaatttttctaaaactcatttagcaacatggcctgaacctgttcacactgcttatggtcagctaactatatttatgtaaatattcatttctctgttgaggaaatgttagtatttgcttttgaggcaacctccagataccatggagggcatgtcatagtcaaagagagggctccctatggtatttctctaaattctggcatttcctttattccaaagcacatctagtgtccccagaagtttgggtagacaattcttggcaacacagagaattacaacatgttcaaaacccaacagcttaatatctaaatcatcaagcaaacatcacatggcaaagggatttctgaatcaaaactgtttcatccttatgatcaacctatggaggtctagcctcgacttacacccattttaccaataagctaagagaagctaagttcctcatcaaggacacaaggctagcatgtgtgagcaagtgacagagttgccctctatgttggttagtgtgccttagccagtgtctcagtaagaaatggagctaaatcaaaacccaaggccaacagccaaaggcacatgagtaacctttgcttggcactgggctcagtttccctggctcctctcagtcctcagttcacagaggcagctgtcatgcaaatagaatccaagcttgttggtcagacctggagataacaaattccatcaaaaatagctcctcatgtgacctagtttgctgtctgttgctatgatacacaccatgaccgaaaagcaaccctggggagagaagggtttatttcatcttacagcttacagttcaccatggaggaaagccaggtgggaacctggaagtggaaattgaagcagagaccagaaaggaatgctgtttactggctggcttagctccttttcttatacagcttaggtctatgtgcccaggggatggtactgccgagcataggctgagcccgcctacatcaaccattagtcaaaaaaaggtccatagacttgcctacaggccaatctcatggaggcaataccccagtggagggtccctcttcgcaggttactctagtttgtgtcaagttgacaaaacctaaccacaaagcacaaacagggtctgcccttgtggcttagccatggatgacactctcagatgatggtgttaccagacaaaccagaggggctcaccaagagtctgccacctaccaaggtagtactctactcctcactgggcaccaacacccatattagctgggccagtacaggacccttgctgtttcctgcatgaattgtccatagaccctgggtctcagcctgccgggagtacctgtaagtagtcgcctcaaacacattattcctgttggaagacttgtctgattctcttttagaactcaatcaacaaacgtttttattttgttttggctttttggagacaagatctctcataggccagcctgacttgaatgtagctgaggatgacctgtgctgctaatcttctcgcctcttcctcccaagtggtaggataataggcataagacaccacagcagttttactccataccagggctctgaacccagactttaaacactctatcaactgattcacattcccaccccatcattcaacaaacatttgaaaaataaaacccttctgccttgagcactctgctaaatacagcctttgagtgcggagtatttcctcacaaccagggtccaagatgaccccatcatacataccacggaaaattaggagatgtttttaggtctctttgcttggggtaatttttatgtgtgtgtgtacacagccctgtgcgtgtgtgtgtgtgtgtgtgtgtgtgtgtacaggcacacacgtgtatgcatgtagaggctacataaaaaccttaggtgtcattctcaggcactctgttcaccccttcacacagcccgaacacacaaaatttgaggcattagcctggagctcaccagttaggctagactgacttgccagcagaccccaggctgtctccatctccccagctctgggattacaaactctatcataccagacatttttatacatattctgagcataaaattcatgtcttcaggctaacaagtcaagagcttaaatgactgagctctcttacgtggtggattttttttaaaactacataatatcttttttttttttttcacttctggggaagaaacaaatgagcctgagtgacaatgcgacagaaaagaaattttgaggagtgtgtgtgtctgtgtgtgtggtggcacatgcctctcatctaatgctagaggctacagtagaatgctcctgaattagtggccagccaaggccaagggctagggttgtaactcagtggcagagggcttgcctagcattcgcaggatttgatccatagcgctataaataataataaataaatacaacagtctaagatgattctccctttcatttatctggatgttatttttgtgttagttttactctgtcatccaatcattgtttgccctatatttggacatttaaaaaaaatctttattccaagtgtgttcaaagctgtatccaaaacctgtccaccaaatgagtccaatgacatacatcttctatattaccatctgttccagatttggctgactcccggcacctgggctgttgctgcacccatgtctcagatagtctagtgatttgagaagtgactagtaattgcaaaatccagactttgtccagaaacttctatgagctccaaaactttcatttacatttctgccagccacaaaccgcttgtgttgtggagagaaccctgtgatgtcttcccacagcatctcagccttgtttcttcccttaaaatattcatcttttcacattagaacatgcaaagggacagtgggagcgaaacccctggactgggacgcacgaagccttcctttctggtcaggctctcactgtagaaacttaggccggtttcagcatgcagtctgctggagaatggctcctgccaacattccaggtctggaagtttgtagtggagttgttgataaccactgttcgccacaggtcttttgtttgtgggtgtcagtgtttctactctcctgacttttatctgaacccaagaaagggaacaatagccttcaagctctctgtgactctgatctgaccagggccacccacactgcagaaggaaacttgcaaagagagacctgcaattctctaagagctccacacagctccaaagacttaggcagcatattttaatctaattattcgtcccccaaccccaccccagaggacagttagacaataaaaggaagattaccagcttagcatcctgtgaacactttgtctgcagctcctacctctgggctctgttagaactagctgtctctcctctctcctaggtggttttcacagccaacgactctggccatcgccactacaccatcgcagccctgctcagcccatactcctacagcaccacggctgtcgtcagcaacccccagaattga

SEQ ID NO: 21 - DNA, 24 bp, Artificial Sequence
  Synthetic
cacagacaatcagacgtaccagta

SEQ ID NO: 22 - DNA, 20 bp, Artificial Sequence
  Synthetic
ccagctttgccagtttacga

SEQ ID NO: 23 - DNA, 18 bp, Artificial Sequence
  Synthetic
ttggacggttgccctctt

SEQ ID NO: 24 - DNA, 22 bp, Artificial Sequence
  Synthetic
gatggcttcccttcgactcttc

SEQ ID NO: 25 - DNA, 25 bp, Artificial Sequence
  Synthetic
cactgacatttctcttgtctcctct

SEQ ID NO: 26 - DNA, 21 bp, Artificial Sequence
  Synthetic
gggctcaccacagatgagaag

SEQ ID NO: 27 - DNA, 20 bp, Artificial Sequence
  Synthetic
cactgttcgccacaggtctt

SEQ ID NO: 28 - DNA, 20 bp, Artificial Sequence
  Synthetic
gctcagcccatactcctaca

SEQ ID NO: 29 - DNA, 18 bp, Artificial Sequence
  Synthetic
gcccaggaggaccaggat

SEQ ID NO: 30 - DNA, 20 bp, Artificial Sequence
  Synthetic
ggcaacttgcttgaggaaga

SEQ ID NO: 31 - DNA, 20 bp, Artificial Sequence
  Synthetic
gcagcaacccagcttcactt

SEQ ID NO: 32 - DNA, 19 bp, Artificial Sequence
  Synthetic
actgagctgggacttgaac

SEQ ID NO: 33 - DNA, 19 bp, Artificial Sequence
  Synthetic
tgcctcactctgagaacca

SEQ ID NO: 34 - DNA, 19 bp, Artificial Sequence
  Synthetic
ggtggagaggctattcggc

SEQ ID NO: 35 - DNA, 18 bp, Artificial Sequence
  Synthetic
ggccgtgcatgtgttcag

SEQ ID NO: 36 - DNA, 23 bp, Artificial Sequence
  Synthetic
ggttcccatttgctcttattcgt

SEQ ID NO: 37 - DNA, 23 bp, Artificial Sequence
  Synthetic
cccacactgcagaaggaaacttg

SEQ ID NO: 38 - DNA, 23 bp, Artificial Sequence
  Synthetic
ggttcccatttgctcttattcgt

SEQ ID NO: 39 - DNA, 22 bp, Artificial Sequence
  Synthetic
ccagcttagcatcctgtgaaca

SEQ ID NO: 40 - DNA, 20 bp, Artificial Sequence
  Synthetic
ggcaacttgcttgaggaaga

SEQ ID NO: 41 - DNA, 22 bp, Artificial Sequence
  Synthetic
tgtggagttcagtagtgtggag

SEQ ID NO: 42 - DNA, 25 bp, Artificial Sequence
  Synthetic
cactgacatttctcttgtctcctct

SEQ ID NO: 43 - DNA, 23 bp, Artificial Sequence
  Synthetic
gggacatctcggtttcctgactt

SEQ ID NO: 44 - DNA, 22 bp, Artificial Sequence
  Synthetic
tccacactactgaactccacaa

SEQ ID NO: 45 - DNA, 21 bp, Artificial Sequence
  Synthetic
cggaacactcgctctacgaaa

SEQ ID NO: 46 - DNA, 18 bp, Artificial Sequence
  Synthetic
gggccagcttcagacaca

SEQ ID NO: 47 - DNA, 22 bp, Artificial Sequence
  Synthetic
cccagggtgctggagaatccaa

SEQ ID NO: 48 - DNA, 22 bp, Artificial Sequence
  Synthetic
gccaagtgtcttccagtacgat

SEQ ID NO: 49 - DNA, 21 bp, Artificial Sequence
  Synthetic
gttccctttcttgggttcaga

SEQ ID NO: 50 - DNA, 23 bp, Artificial Sequence
  Synthetic
gatgctactgctttggcaagatc

SEQ ID NO: 51 - DNA, 20 bp, Artificial Sequence
  Synthetic
cctgagctgctaacacggtt

SEQ ID NO: 52 - DNA, 23 bp, Artificial Sequence
  Synthetic
agctacagaccatgcttagtgta

SEQ ID NO: 53 - DNA, 24 bp, Artificial Sequence
  Synthetic
tgccagtttaggaggaatatgttc

SEQ ID NO: 54 - DNA, 25 bp, Artificial Sequence
  Synthetic
ctgaggaaacagaggtaccagatat

SEQ ID NO: 55 - DNA, 24 bp, Artificial Sequence
  Synthetic
agtcacacagttctgtcaaatcag

SEQ ID NO: 56 - DNA, 17 bp, Artificial Sequence
  Synthetic
gaacacggcggcatcag

SEQ ID NO: 57 - DNA, 20 bp, Artificial Sequence
  Synthetic
tcctgtgggagggttctttg

SEQ ID NO: 58 - DNA, 20 bp, Artificial Sequence
  Synthetic
ccctctctctgagccctcta

SEQ ID NO: 59 - DNA, 21 bp, Artificial Sequence
  Synthetic
gctgcctaagtctttggagct

SEQ ID NO: 60 - DNA, 20 bp, Artificial Sequence
  Synthetic
ccctctctctgagccctcta

SEQ ID NO: 61 - DNA, 25 bp, Artificial Sequence
  Synthetic
gagaggagagacagctagttctaac

SEQ ID NO: 62 - DNA, 23 bp, Artificial Sequence
  Synthetic
agctacagaccatgcttagtgta

SEQ ID NO: 63 - DNA, 22 bp, Artificial Sequence
  Synthetic
gccctcttcatacaggaatcac

SEQ ID NO: 64 - DNA, 19 bp, Artificial Sequence
  Synthetic
cggacagcatccaggactt

SEQ ID NO: 65 - DNA, 26 bp, Artificial Sequence
  Synthetic
tcatgtaatctggcttcagagtggga

SEQ ID NO: 66 - DNA, 27 bp, Artificial Sequence
  Synthetic
tgggaggcaattcttagtttcaatgga

SEQ ID NO: 67 - DNA, 23 bp, Artificial Sequence
  Synthetic
tcccaaaggtgtctgtctgcaca

SEQ ID NO: 68 - DNA, 22 bp, Artificial Sequence
  Synthetic
ctcctttgcctcgctggactgg

SEQ ID NO: 69 - DNA, 19 bp, Artificial Sequence
  Synthetic
cggacagcatccaggactt

SEQ ID NO: 70 - DNA, 29 bp, Artificial Sequence
  Synthetic
agaaggagtgtacagagtagaactggaca

SEQ ID NO: 71 - DNA, 27 bp, Artificial Sequence
  Synthetic
tgtttgtgggtgtcagtgtttctactc

SEQ ID NO: 72 - DNA, 21 bp, Artificial Sequence
  Synthetic
caccacggctgtcgtcagcaa

SEQ ID NO: 73 - DNA, 23 bp, Artificial Sequence
  Synthetic
cttgccaaagcagtagcatccca

SEQ ID NO: 74 - DNA, 23 bp, Artificial Sequence
  Synthetic
aggtcagaaagcagagtggacca

SEQ ID NO: 75 - DNA, 23 bp, Artificial Sequence
  Synthetic
cccaggcaattcctaccttccca

SEQ ID NO: 76 - DNA, 28 bp, Artificial Sequence
  Synthetic
tctgagcattctacctcattgctttggt

SEQ ID NO: 77 - DNA, 23 bp, Artificial Sequence
  Synthetic
aggctgtcccagcacctgagtcg

SEQ ID NO: 78 - DNA, 23 bp, Artificial Sequence
  Synthetic
tgggcacaacagacaatcggctg

SEQ ID NO: 79 - DNA, 23 bp, Artificial Sequence
  Synthetic
aaggctgctgatgacacctggga

SEQ ID NO: 80 - DNA, 27 bp, Artificial Sequence
  Synthetic
agattcagacacacacaacttaccagc

SEQ ID NO: 81 - DNA, 28 bp, Artificial Sequence
  Synthetic
agacctgcaattctctaagagctccaca

SEQ ID NO: 82 - DNA, 27 bp, Artificial Sequence
  Synthetic
agattcagacacacacaacttaccagc

SEQ ID NO: 83 - DNA, 24 bp, Artificial Sequence
  Synthetic
ttgtctgcagctcctacctctggg

SEQ ID NO: 84 - DNA, 23 bp, Artificial Sequence
  Synthetic
aggtcagaaagcagagtggacca

SEQ ID NO: 85 - DNA, 29 bp, Artificial Sequence
  Synthetic
ttgacatgtgtgggtgagagattttactg

SEQ ID NO: 86 - DNA, 22 bp, Artificial Sequence
  Synthetic
cccagggtgctggagaatccaa

SEQ ID NO: 87 - RNA, 16 nt, Artificial Sequence
  Synthetic
guuuuagagcuaugcu

SEQ ID NO: 88 - RNA, 67 nt, Artificial Sequence
  Synthetic
agcauagcaaguuaaaauaaggcuaguccguuaucaacuugaaaaaguggcaccgagucggugcuuu

SEQ ID NO: 89 - RNA, 77 nt, Artificial Sequence
  Synthetic
guuuuagagcuagaaauagcaaguuaaaauaaggcuaguccguuaucaacuugaaaaaguggcaccgagucggugcu

SEQ ID NO: 90 - DNA, 444 bp, Artificial Sequence
  Synthetic
atggcttctcatcgtctgctcctcctctgccttgctggactggtatttgtgtctgaggctggccctacgggcaccggtgaatccaagtgtcctctgatggtcaaagttctagatgctgtccgaggcagtcctgccatcaatgtggccgtgcatgtgttcagaaaggctgctgatgacacctgggagccatttgcctctgggaaaaccagtgagtctggagagctgcatgggctcacaactgaggaggaatttgtagaagggatatacaaagtggaaatagacaccaaatcttactggaaggcacttggcatctccccattccatgagcatgcagaggtggtattcacagccaacgactccggcccccgccgctacaccattgccgccctgctgagcccctactcctattccaccacggctgtcgtcaccaatcccaaggaatga

SEQ ID NO: 91 - DNA, 444 bp, Artificial Sequence
  Synthetic
atggcttcccttcgactcttcctcctttgcctcgctggactggtatttgtgtctgaagctggccccgcgggcaccggtgaatccaagtgtcctctgatggtcaaagttctagatgctgtccgaggcagtcctgccatcaatgtggccgtgcatgtgttcagaaaggctgctgatgacacctgggagccatttgcctctgggaaaaccagtgagtctggagagctgcatgggctcacaactgaggaggaatttgtagaagggatatacaaagtggaaatagacaccaaatcttactggaaggcacttggcatctccccattccatgagcatgcagaggtggtattcacagccaacgactccggcccccgccgctacaccattgccgccctgctgagcccctactcctattccaccacggctgtcgtcaccaatcccaaggaatga

SEQ ID NO: 92 - DNA, 444 bp, Artificial Sequence
  Synthetic
atggcttcccttcgactcttcctcctttgcctcgctggactggtatttgtgtctgaagctggccccgcgggtgctggagaatccaaatgtcctctgatggtcaaagtcctggatgctgtccgaggcagccctgctgtagacgtggctgtaaaagtgttcaaaaagacctctgagggatcctgggagccctttgcctctgggaagaccgcggagtctggagagctgcacgggctcaccacagatgagaagtttgtagaaggagtgtacagagtagaactggacaccaaatcgtactggaagacacttggcatttccccgttccatgaattcgcggatgtggttttcacagccaacgactctggccatcgccactacaccatcgcagccctgctcagcccatactcctacagcaccacggctgtcgtcagcaacccccagaattga

SEQ ID NO: 93 - DNA, 4176 bp, Artificial Sequence
  Synthetic
  misc_feature (1)..(3): Start Codon
  misc_feature (10)..(30): 5' NLS
  misc_feature (4126)..(4173): 3' NLS
  misc_feature (4174)..(4176): Stop Codon
atggacaagcccaagaaaaagcggaaagtgaagtacagcatcggcctggacatcggcaccaactctgtgggctgggccgtgatcaccgacgagtacaaggtgcccagcaagaaattcaaggtgctgggcaacaccgacaggcacagcatcaagaagaacctgatcggcgccctgctgttcgacagcggcgaaacagccgaggccaccagactgaagagaaccgccagaagaagatacaccaggcggaagaacaggatctgctatctgcaagagatcttcagcaacgagatggccaaggtggacgacagcttcttccacagactggaagagtccttcctggtggaagaggacaagaagcacgagagacaccccatcttcggcaacatcgtggacgaggtggcctaccacgagaagtaccccaccatctaccacctgagaaagaaactggtggacagcaccgacaaggccgacctgagactgatctacctggccctggcccacatgatcaagttcagaggccacttcctgatcgagggcgacctgaaccccgacaacagcgacgtggacaagctgttcatccagctggtgcagacctacaaccagctgttcgaggaaaaccccatcaacgccagcggcgtggacgccaaggctatcctgtctgccagactgagcaagagcagaaggctggaaaatctgatcgcccagctgcccggcgagaagaagaacggcctgttcggcaacctgattgccctgagcctgggcctgacccccaacttcaagagcaacttcgacctggccgaggatgccaaactgcagctgagcaaggacacctacgacgacgacctggacaacctgctggcccagatcggcgaccagtacgccgacctgttcctggccgccaagaacctgtctgacgccatcctgctgagcgacatcctgagagtgaacaccgagatcaccaaggcccccctgagcgcctctatgatcaagagatacgacgagcaccaccaggacctgaccctgctgaaagctctcgtgcggcagcagctgcctgagaagtacaaagaaatcttcttcgaccagagcaagaacggctacgccggctacatcgatggcggcgctagccaggaagagttctacaagttcatcaagcccatcctggaaaagatggacggcaccgaggaactgctcgtgaagctgaacagagaggacctgctgagaaagcagagaaccttcgacaacggcagcatcccccaccagatccacctgggagagctgcacgctatcctgagaaggcaggaagatttttacccattcctgaaggacaaccgggaaaagatcgagaagatcctgaccttcaggatcccctactacgtgggccccctggccagaggcaacagcagattcgcctggatgaccagaaagagcgaggaaaccatcaccccctggaacttcgaggaagtggtggacaagggcgccagcgcccagagcttcatcgagagaatgacaaacttcgataagaacctgcccaacgagaaggtgctgcccaagcacagcctgctgtacgagtacttcaccgtgtacaacgagctgaccaaagtgaaatacgtgaccgagggaatgagaaagcccgccttcctgagcggcgagcagaaaaaggccatcgtggacctgctgttcaagaccaacagaaaagtgaccgtgaagcagctgaaagaggactacttcaagaaaatcgagtgcttcgactccgtggaaatctccggcgtggaagatagattcaacgcctccctgggcacataccacgatctgctgaaaattatcaaggacaaggacttcctggataacgaagagaacgaggacattctggaagatatcgtgctgaccctgacactgtttgaggaccgcgagatgatcgaggaaaggctgaaaacctacgctcacctgttcgacgacaaagtgatgaagcagctgaagagaaggcggtacaccggctggggcaggctgagcagaaagctgatcaacggcatcagagacaagcagagcggcaagacaatcctggatttcctgaagtccgacggcttcgccaaccggaacttcatgcagctgatccacgacgacagcctgacattcaaagaggacatccagaaagcccaggtgtccggccagggcgactctctgcacgagcatatcgctaacctggccggcagccccgctatcaagaagggcatcctgcagacagtgaaggtggtggacgagctcgtgaaagtgatgggcagacacaagcccgagaacatcgtgatcgagatggctagagagaaccagaccacccagaagggacagaagaactcccgcgagaggatgaagagaatcgaagagggcatcaaagagctgggcagccagatcctgaaagaacaccccgtggaaaacacccagctgcagaacgagaagctgtacctgtactacctgcagaatggccgggatatgtacgtggaccaggaactggacatcaacagactgtccgactacgatgtggaccatatcgtgcctcagagctttctgaaggacgactccatcgataacaaagtgctgactcggagcgacaagaacagaggcaagagcgacaacgtgccctccgaagaggtcgtgaagaagatgaagaactactggcgacagctgctgaacgccaagctgattacccagaggaagttcgataacctgaccaaggccgagagaggcggcctgagcgagctggataaggccggcttcatcaagaggcagctggtggaaaccagacagatcacaaagcacgtggcacagatcctggactcccggatgaacactaagtacgacgaaaacgataagctgatccgggaagtgaaagtgatcaccctgaagtccaagctggtgtccgatttccggaaggatttccagttttacaaagtgcgcgagatcaacaactaccaccacgcccacgacgcctacctgaacgccgtcgtgggaaccgccctgatcaaaaagtaccctaagctggaaagcgagttcgtgtacggcgactacaaggtgtacgacgtgcggaagatgatcgccaagagcgagcaggaaatcggcaaggctaccgccaagtacttcttctacagcaacatcatgaactttttcaagaccgaaatcaccctggccaacggcgagatcagaaagcgccctctgatcgagacaaacggcgaaaccggggagatcgtgtgggataagggcagagacttcgccacagtgcgaaaggtgctgagcatgccccaagtgaatatcgtgaaaaagaccgaggtgcagacaggcggcttcagcaaagagtctatcctgcccaagaggaacagcgacaagctgatcgccagaaagaaggactgggaccccaagaagtacggcggcttcgacagccctaccgtggcctactctgtgctggtggtggctaaggtggaaaagggcaagtccaagaaactgaagagtgtgaaagagctgctggggatcaccatcatggaaagaagcagctttgagaagaaccctatcgactttctggaagccaagggctacaaagaagtgaaaaaggacctgatcatcaagctgcctaagtactccctgttcgagctggaaaacggcagaaagagaatgctggcctctgccggcgaactgcagaagggaaacgagctggccctgcctagcaaatatgtgaacttcctgtacctggcctcccactatgagaagctgaagggcagccctgaggacaacgaacagaaacagctgtttgtggaacagcataagcactacctggacgagatcatcgagcagatcagcgagttctccaagagagtgatcctggccgacgccaatctggacaaggtgctgtctgcctacaacaagcacagggacaagcctatcagagagcaggccgagaatatcatccacctgttcaccctgacaaacctgggcgctcctgccgccttcaagtactttgacaccaccatcgaccggaagaggtacaccagcaccaaagaggtgctggacgccaccctgatccaccagagcatcaccggcctgtacgagacaagaatcgacctgtctcagctgggaggcgacaagagacctgccgccactaagaaggccggacaggccaaaaagaagaagtga

SEQ ID NO: 94 - protein, 1391 aa, Artificial Sequence
  Synthetic
  MISC_FEATURE (4)..(10): 5' NLS
  MISC_FEATURE (1376)..(1391): 3' NLS
MDKPKKKRKVKYSIGLDIGTNSVGWAVITDEYKVPSKKFKVLGNTDRHSIKKNLIGALLFDSGETAEATRLKRTARRRYTRRKNRICYLQEIFSNEMAKVDDSFFHRLEESFLVEEDKKHERHPIFGNIVDEVAYHEKYPTIYHLRKKLVDSTDKADLRLIYLALAHMIKFRGHFLIEGDLNPDNSDVDKLFIQLVQTYNQLFEENPINASGVDAKAILSARLSKSRRLENLIAQLPGEKKNGLFGNLIALSLGLTPNFKSNFDLAEDAKLQLSKDTYDDDLDNLLAQIGDQYADLFLAAKNLSDAILLSDILRVNTEITKAPLSASMIKRYDEHHQDLTLLKALVRQQLPEKYKEIFFDQSKNGYAGYIDGGASQEEFYKFIKPILEKMDGTEELLVKLNREDLLRKQRTFDNGSIPHQIHLGELHAILRRQEDFYPFLKDNREKIEKILTFRIPYYVGPLARGNSRFAWMTRKSEETITPWNFEEVVDKGASAQSFIERMTNFDKNLPNEKVLPKHSLLYEYFTVYNELTKVKYVTEGMRKPAFLSGEQKKAIVDLLFKTNRKVTVKQLKEDYFKKIECFDSVEISGVEDRFNASLGTYHDLLKIIKDKDFLDNEENEDILEDIVLTLTLFEDREMIEERLKTYAHLFDDKVMKQLKRRRYTGWGRLSRKLINGIRDKQSGKTILDFLKSDGFANRNFMQLIHDDSLTFKEDIQKAQVSGQGDSLHEHIANLAGSPAIKKGILQTVKVVDELVKVMGRHKPENIVIEMARENQTTQKGQKNSRERMKRIEEGIKELGSQILKEHPVENTQLQNEKLYLYYLQNGRDMYVDQELDINRLSDYDVDHIVPQSFLKDDSIDNKVLTRSDKNRGKSDNVPSEEVVKKMKNYWRQLLNAKLITQRKFDNLTKAERGGLSELDKAGFIKRQLVETRQITKHVAQILDSRMNTKYDENDKLIREVKVITLKSKLVSDFRKDFQFYKVREINNYHHAHDAYLNAVVGTALIKKYPKLESEFVYGDYKVYDVRKMIAKSEQEIGKATAKYFFYSNIMNFFKTEITLANGEIRKRPLIETNGETGEIVWDKGRDFATVRKVLSMPQVNIVKKTEVQTGGFSKESILPKRNSDKLIARKKDWDPKKYGGFDSPTVAYSVLVVAKVEKGKSKKLKSVKELLGITIMERSSFEKNPIDFLEAKGYKEVKKDLIIKLPKYSLFELENGRKRMLASAGELQKGNELALPSKYVNFLYLASHYEKLKGSPEDNEQKQLFVEQHKHYLDEIIEQISEFSKRVILADANLDKVLSAYNKHRDKPIREQAENIIHLFTLTNLGAPAAFKYFDTTIDRKRYTSTKEVLDATLIHQSITGLYETRIDLSQLGGDKRPAATKKAGQAKKKK